European Patent Application EP 4 524 250 A1, published March 19, 2025. Title: 包含UTR的核酸构建体及其应用. Applicant: 上海瑞宏迪医药有限公司. The sequence listing filed with the application follows.

SEQUENCE LISTING (131 sequences)

SEQ ID NO: 1 - DNA, 517 bp, synthetic construct
  source 1..517: mol_type = other DNA; note = B1 (ACTG1 3'UTR)
ccgactacctcatgaagatcctcactgagcgaggctacagcttcaccaccacggccgagcgggaaatcgtgcgcgacatcaaggagaagctgtgctacgtcgccctggacttcgagcaggagatggccaccgccgcatcctcctcttctctggagaagagctacgagctgcccgatggccaggtcatcaccattggcaatgagcggttccggtgtccggaggcgctgttccagccttccttcctgggtatggaatcttgcggcatccacgagaccaccttcaactccatcatgaagtgtgacgtggacatccgcaaagacctgtacgccaacacggtgctgtcgggcggcaccaccatgtacccgggcattgccgacaggatgcagaaggagatcaccgccctggcgcccagcaccatgaagatcaagatcatcgcacccccagagcgcaagtactcggtgtggatcggtggctccatcctggcctcactgtccaccttccagcagatgtggattag

SEQ ID NO: 2 - DNA, 282 bp, synthetic construct
  source 1..282: mol_type = other DNA; note = B2 (ATP6V0B)
atgatatgtgtgggtggggccgtgcctcacttttatttattgctggttttcctgggacagctggagctgtgtcccttagcctttcagaggcttggtgttcagggccctccctgcactcccctcttgctgcgtgttgatttggaggcactgcagtccaggccgagtcctcagtgcggggagcaggctgctgctgctgactctgtgcagctgcgcacctgtgtcccccacctccaccctcaacccatcttcctagtgtttgtgaaataaacttggtatttgtct

SEQ ID NO: 3 - DNA, 308 bp, synthetic construct
  source 1..308: mol_type = other DNA; note = B3 (ATP6V0B)
gttgaagaacttctctctaccgagcagcccgtaaccccctttttctccctcactgctgcaggagtctgctacaccatttttgatttgggcttccgctttgatgtggcatggttcctgacggagacttcgcccttcatgtggtccaacctgggcattggcctagctatctccctgtctgtggttggggcagcctggggcatctatattaccggctcctccatcattggtggaggagtgaaggcccccaggatcaagaccaagaacctggtcagcatcatcttctgtgaggctgtggccatctacggcat

SEQ ID NO: 4 - DNA, 226 bp, synthetic construct
  source 1..226: mol_type = other DNA; note = B4 (ATP6V0E1 3'UTR)
ggaagaagacatgctctacagtgctcagtctttgaggtgactatgcttgtgacctttcttatcagtatggtcaggcagtcagagtttgccttgactttttctcacattttatggccattttaacacgtggcaagggcaagctgctgaatgcaaacacgatctgaagagcagaaataaaattggaacttaagccttagcttacctaaatctcattaagattcttttt

SEQ ID NO: 5 - DNA, 461 bp, synthetic construct
  source 1..461: mol_type = other DNA; note = B5 (ATP6V0E1 3'UTR)
atgcaaaatcacctccaaaccagaccacttttcttgacttgcctgttttggccattagctgccttaaacgttaacagcacatttgaatgccttattctacaatgcagcgtgttttcctttgccttttttgcactttggtgaattacgtgcctccataacctgaactgtgccgactccacaaaacgattatgtactcttctgagatagaagatgctgttcttctgagagatacgttactctctccttggaatctgtggatttgaagatggctcctgccttctcacgtgggaatcagtgaagtgtttagaaactgctgcaagacaaacaagactccagtggggtggtcagtaggagagcacgttcagagggaagagccatctcaacagaatcgcaccaaactatactttcaggatgaatttcttctttctgccatcttttggaataaatattttcctcctttc

SEQ ID NO: 6 - DNA, 499 bp, synthetic construct
  source 1..499: mol_type = other DNA; note = B6 (CFL1 3'UTR)
gccccttctggccccctgcctggagcatctggcagccccacacctgcccttgggggttgcaggctgcccccttcctgccagaccggaggggctggggggatcccagcagggggagggcaatcccttcaccccagttgccaaacagaccccccaccccctggattttccttctccctccatcccttgacggttctggccttcccaaactgcttttgatcttttgattcctcttgggctgaagcagaccaagttccccccaggcaccccagttgtgggggagcctgtattttttttaacaacatccccattccccacctggtcctcccccttcccatgctgccaacttctaaccgcaatagtgactctgtgcttgtctgtttagttctgtgtataaatggaatgttgtggagatgacccctccctgtgccggctggttcctctcccttttcccctggtcacggctactcatggaagcaggaccagtaagggaccttcgatt

SEQ ID NO: 7 - DNA, 282 bp, synthetic construct
  source 1..282: mol_type = other DNA; note = B7 (CFL1 3'UTR)
gccccttctggccccctgcctggagcatctggcagccccacacctgcccttgggggttgcaggctgcccccttcctgccagaccggaggggctggggggatcccagcagggggagggcaatcccttcaccccagttgccaaacagaccccccaccccctggattttccttctccctccatcccttgacggttctggccttcccaaactgcttttgatcttttgattcctcttgggctgaagcagaccaagttccccccaggcaccccagttgtgggggagcc

SEQ ID NO: 8 - DNA, 361 bp, synthetic construct
  source 1..361: mol_type = other DNA; note = B8 (CFL1 3'UTR)
gccccttctggccccctgcctggagcatctggcagccccacacctgcccttgggggttgcaggctgcccccttcctgccagaccggaggggctggggggatcccagcagggggagggcaatcccttcaccccagttgccaaacagaccccccaccccctggattttccttctccctccatcccttgacggttctggccttcccaaactgcttttgatcttttgattcctcttgggctgaagcagaccaagttccccccaggcaccccagttgtgggggagcctgtattttttttaacaacatccccattccccacctggtcctcccccttcccatgctgccaacttctaaccgcaatagtg

SEQ ID NO: 9 - DNA, 128 bp, synthetic construct
  source 1..128: mol_type = other DNA; note = B9 (COX4I1 3'UTR)
gagatgctggcctgcgcctgcacctgcgcctggctctgtcaccgccatgcaactccatgcctatttactggaaacctgttatgccaaacagttgtaccactgctaataaatgaccagtttacctgaaa

SEQ ID NO: 10 - DNA, 319 bp, synthetic construct
  source 1..319: mol_type = other DNA; note = B10 (COX4I1 3'UTR)
agggacccacaggcgcgcccagcagctctcggaagcgttgtatcgcattaagttcaaggagagctttgctgagatgaacaggggctcgaacgagtggaagacggttgtgggcggtgccatgttcttcatcggtttcaccgcgctcgttatcatgtggcagaagcactatgggcttagcctccaagtgggactacgaaaagaacgagtggaagaagtgagagatgctggcctgcgcctgcacctgcgcctggctctgtcaccgccatgcaactccatgcctatttactggaaacctgttatgccaaacagttgtaccact

SEQ ID NO: 11 - DNA, 303 bp, synthetic construct
  source 1..303: mol_type = other DNA; note = B11 (COX4I1 3'UTR)
agaggaccttctgcttttagcttattttgttgctaactttttacaaacaaagggctaattttaaaatgtcagtgttgtcagtggtcagaaaccgtgtgtttgagcgggtgttgagtggcaggtggctctgctgacctggtggctggtgtgtcgggaggatttaacctgtgtgagggattggcctagaaacaacctgttgagatagtcttgccccataacctgtctcacaccgtagtgtacggccccctcccgcaaagctttgacaaagagtgggtggccaagcagaccaagaggatgctggac

SEQ ID NO: 12 - DNA, 232 bp, synthetic construct
  source 1..232: mol_type = other DNA; note = B12 (CTSB 3'UTR)
tctgccgtgggcctgtcgtgccagtcctgggggcgagatcgggagaatcacgtcctggaactgcatgttcttgcgactcttgggacttcatcttaacttctcgctgccccagccatgttttcaaccatggcatccctcccccaattagttccctgtcatcctcgtcaaccttctctgtaagtgcctggtaagcttgcccttgcttaagaactcaaaacatagctgtgctcta

SEQ ID NO: 13 - DNA, 115 bp, synthetic construct
  source 1..115: mol_type = other DNA; note = B13 (FAM166A 3'UTR)
aaatgctttaatggtggtgtctgtacagcatggatgtggacagggaaaacagcaagtgcacacagtgggacaggccacaggacaggctgggagtgaataaagagttcacactgct

SEQ ID NO: 14 - DNA, 196 bp, synthetic construct
  source 1..196: mol_type = other DNA; note = B14 (NDUFB9 3'UTR)
tatctaagtgtatcaatttaacatttataatcaccttacaagtaagttaaagtgcattccctggtcgttttggctttgtctttgattttgcttcagatctccttctctttagtcctttgtctgacttttttgccttcttgctatactttccctcaacctgcctctccactattttcttaggcatttttcagtcatg

SEQ ID NO: 15 - DNA, 54 bp, synthetic construct
  source 1..54: mol_type = other DNA; note = A1 (ACTG1 5'UTR)
ctctcgcactctgttcttccgccgctccgccgtcgcgtttctctgccggtcgca

SEQ ID NO: 16 - DNA, 185 bp, synthetic construct
  source 1..185: mol_type = other DNA; note = A2 (ATP6V0B 5'UTR)
gggcgggcggacagactgcgggacggacggtggacgctgggacgcgtttgtagctccggccccgccgttccgacccccgccgccgtcgccgccatgacggggctagcactgctctactccggggtcttcgtggccttctgggcctgcgcgctggccgtgggttcctgacggagacttcgcccttc

SEQ ID NO: 17 - DNA, 81 bp, synthetic construct
  source 1..81: mol_type = other DNA; note = A3 (ATP6V0B 5'UTR)
agactgcgggacggacggtggacgctgggacgcgtttgtagctccggccccgccgttccgacccccgccgccgtcgccgcc

SEQ ID NO: 18 - DNA, 30 bp, synthetic construct
  source 1..30: mol_type = other DNA; note = A4 (ATP6V0E1 5'UTR)
ggggtaggggttggcgctcaggcggcgacc

SEQ ID NO: 19 - DNA, 80 bp, synthetic construct
  source 1..80: mol_type = other DNA; note = A5 (ATP6V0E1 5'UTR)
gtcacgcggtcagctattgacacttcctggtgggatccgagtgaggcgacggggtaggggttggcgctcaggcggcgacc

SEQ ID NO: 20 - DNA, 234 bp, synthetic construct
  source 1..234: mol_type = other DNA; note = A6 (CFL1 5'UTR)
ggccggcgggaagactccgttacccagcgagcgaggcggcggcgcagggccagcggactccatttcccgtcggctcgcggtgggagcgccggaagcccgccccacccctcattgtgcggctcctactaaacggaaggggccgggagaggccgcgttcagtcgggtcccggcagcggctgcagcgctctcgtcttctgcggctctcggtgccctctccttttcgtttccggaaac

SEQ ID NO: 21 - DNA, 128 bp, synthetic construct
  source 1..128: mol_type = other DNA; note = A7 (CFL1 5'UTR)
ctcctggctcgggcaccccgaagcacgacgcagagtaggaagagtttaaagacctcgaggcctctgggcacttgagtttggcctccggtgtggctgtctctgatggtgtcatcaaggtgttcaacgac

SEQ ID NO: 22 - DNA, 151 bp, synthetic construct
  source 1..151: mol_type = other DNA; note = A8 (CFL1 5'UTR)
acgtggccggcttcttctgcagttccggggagtttgggggaccagatttaccttggattgcccctccctctcctggctcgggcaccccgaagcacgacgcagagcctccggtgtggctgtctctgatggtgtcatcaaggtgttcaacgac

SEQ ID NO: 23 - DNA, 70 bp, synthetic construct
  source 1..70: mol_type = other DNA; note = A9 (COX4I1 5'UTR)
gcggccttgctctcttccggtcgcgggacaccgggtgtagagggcggtcgcggcgggcagtggcggcaga

SEQ ID NO: 24 - DNA, 46 bp, synthetic construct
  source 1..46: mol_type = other DNA; note = A10 (COX4I1 5'UTR)
gggacaccgggtgtagagggcggtcgcggcgggcagtggcggcaga

SEQ ID NO: 25 - DNA, 71 bp, synthetic construct
  source 1..71: mol_type = other DNA; note = A11 (COX4I1 5'UTR)
cgcggccttgctctcttccggtcgcgggacaccgggtgtagagggcggtcgcggcgggcagtggcggcaga

SEQ ID NO: 26 - DNA, 137 bp, synthetic construct
  source 1..137: mol_type = other DNA; note = A12 (CTSB 5'UTR)
ggccggggctggcccaggctacggcggctgcagggctccggcaaccgctccggcaacgccaaccgctccgctgcgcgcaggctgggctgcaggctctcggctgcagcgctgggtggatctaggatccggcttccaac

SEQ ID NO: 27 - DNA, 55 bp, synthetic construct
  source 1..55: mol_type = other DNA; note = A13 (FAM166A 5'UTR)
aagggagctggatgccgggagggactggagccagcaaggccagagtgaaagcaaa

SEQ ID NO: 28 - DNA, 56 bp, synthetic construct
  source 1..56: mol_type = other DNA; note = A14 (NDUFB9 5'UTR)
gcagcaggcgtgcagtttcccggctctccgcgcggccggggaaggtcagcgccgta

SEQ ID NO: 29 - DNA, 68 bp, synthetic construct
  source 1..68: mol_type = other DNA; note = A15 (CHCHD10 5'UTR)
ggcatttgtccccgcgacagcaccgctgccgccgtctctaaggtcgcccgggtcccaccgccgccacc

SEQ ID NO: 30 - DNA, 46 bp, synthetic construct
  source 1..46: mol_type = other DNA; note = A16 (CHCHD10 5'UTR)
ccgctgccgccgtctctaaggtcgcccgggtcccaccgccgccacc

SEQ ID NO: 31 - DNA, 41 bp, synthetic construct
  source 1..41: mol_type = other DNA; note = A17 (SLC38A2 5'UTR)
atgtcttttttgtgtgtttgttttcatggtattcctatgaa

SEQ ID NO: 32 - DNA, 48 bp, synthetic construct
  source 1..48: mol_type = other DNA; note = A18 (NDUFA11 5'UTR)
gcttcccgagctggcggggtccgtggtgcgggatcgagattgcgggct

SEQ ID NO: 33 - DNA, 69 bp, synthetic construct
  source 1..69: mol_type = other DNA; note = A19 (NDUFV3 5'UTR)
ggcggctgttcaggcgcgggtgcgcgcgcagctgctgtggccctgcttggtgcgcccgctgtcaccgcc

SEQ ID NO: 34 - DNA, 128 bp, synthetic construct
  source 1..128: mol_type = other DNA; note = A20 (PRDX5 5'UTR)
cgcgcctgcgcagtggaggcggcccaggcccgccttccgcagggtgtcgccgctgtgccgctagcggtgccccgcctgctgcggtggcaccagccaggaggcggagtggaagtggccgtggggcgggt

SEQ ID NO: 35 - DNA, 59 bp, synthetic construct
  source 1..59: mol_type = other DNA; note = A21 (GUK1 5'UTR)
cagcagatggggactagaggccgcactgctatccacagcctctcttctcacccccaggc

SEQ ID NO: 36 - DNA, 68 bp, synthetic construct
  source 1..68: mol_type = other DNA; note = A22 (GUK1 5'UTR)
gctggccgggctggctgcggccgccctgggccgggccccaccggacgcctctcttctcacccccaggc

SEQ ID NO: 37 - DNA, 96 bp, synthetic construct
  source 1..96: mol_type = other DNA; note = A23 (GUK1 5'UTR)
agaggtggccccggatgctgcggcgcccgctggccgggctggctgcggccgccctgggccgggccccaccggacgcctctcttctcacccccaggc

SEQ ID NO: 38 - DNA, 37 bp, synthetic construct
  source 1..37: mol_type = other DNA; note = A24 (IAH1 5'UTR)
tggctggcggccccgccccgccccgcccggctgctcc

SEQ ID NO: 39 - DNA, 59 bp, synthetic construct
  source 1..59: mol_type = other DNA; note = A25 (ABHD16A 5'UTR)
ggagggcggggccggcagggggacctgctgctggaagagcagcggcccgagccggggcc

SEQ ID NO: 40 - DNA, 132 bp, synthetic construct
  source 1..132: mol_type = other DNA; note = A26 (SLC25A39 5'UTR)
tttcggcgtcggcctaggtgcgctgcgagcgcgcgcggaccgcgcacaggcggcggagccggtatgggcccgcctgaccctgggcgccgcgccgcacgagcaccagcctagagccaggactgaagcttcaag

SEQ ID NO: 41 - DNA, 51 bp, synthetic construct
  source 1..51: mol_type = other DNA; note = A27 (ATPIF1 5'UTR)
cgagagactgcttgctgcggcagagacgccagaggtgcagctccagcagca

SEQ ID NO: 42 - DNA, 71 bp, synthetic construct
  source 1..71: mol_type = other DNA; note = A28 (ANAPC11 5'UTR)
cggagtttcgtcatgttggccaggcccatttgagatctttgaagatatcctcaacgtgaggctctgctgcc

SEQ ID NO: 43 - DNA, 55 bp, synthetic construct
  source 1..55: mol_type = other DNA; note = A29 (ANAPC11 5'UTR)
gggcgcggcttcggcgggcggcagccgctgcagacgagctgcgggctctgctgcc

SEQ ID NO: 44 - DNA, 48 bp, synthetic construct
  source 1..48: mol_type = other DNA; note = A30 (CCDC12 5'UTR)
gcctgcgcgatgcaagacgggagaaaaggaggggcgtacgcgggcaag

SEQ ID NO: 45 - DNA, 132 bp, synthetic construct
  source 1..132: mol_type = other DNA; note = A31 (MRPL14 5'UTR)
atcgcgtccgccgggctgggcctggcgcgcaggcgctaggaagaggccgcgtggggcgaaggcggcgcttggctggtggggcccgcggcgggattttcccgggcggcgagagcggatctatcttgggatccc

SEQ ID NO: 46 - DNA, 27 bp, synthetic construct
  source 1..27: mol_type = other DNA; note = A32 (APOA1BP 5'UTR)
gccgggggcgcgcgctctgcgagctgg

SEQ ID NO: 47 - DNA, 43 bp, synthetic construct
  source 1..43: mol_type = other DNA; note = A33 (APOA1BP 5'UTR)
gccggggccgggccgggccgggggcgcgcgctctgcgagctgg

SEQ ID NO: 48 - DNA, 47 bp, synthetic construct
  source 1..47: mol_type = other DNA; note = Mod. 5'UTR
gggaaataagagagaaaagaagagtaagaagaaatataagagccacc

SEQ ID NO: 49 - DNA, 119 bp, synthetic construct
  source 1..119: mol_type = other DNA; note; note (original language) = a-球蛋白 3'UTR
tgataataggctggagcctcggtggccatgcttcttgccccttgggcctccccccagcccctcctccccttcctgcacccgtacccccgtggtctttgaataaagtctgagtgggcggc

SEQ ID NO: 50 - RNA, 52 nt, synthetic construct
  source 1..52: mol_type = other RNA; note; note (original language) = a-1 球蛋白 5'UTR
agacgaactagtattcttctggtccccacagactcagagagaacccgccacc

SEQ ID NO: 51 - DNA, 317 bp, synthetic construct
  source 1..317: mol_type = other DNA; note = haplogroup U8b1b1 mitochondrion 3'UTR
ctcgagctggtactgcatgcacgcaatgctagctgcccctttcccgtcctgggtaccccgagtctcccccgacctcgggtcccaggtatgctcccacctccacctgccccactcaccacctctgctagttccagacacctgctatactaatcgctagccgcgtcgctccccagggttggtcaatttcgtgccagccacaccgagacctggtccagagcccaagcacgccacacccccacgggaaacagcagtgattaacctttagcaataaacgaaagtttaactaacagcaatgcagctcaaaacgcttagcctag

SEQ ID NO: 52 - DNA, 110 bp, synthetic construct
  source 1..110: mol_type = other DNA; note = A30L70 PolyA
aaaaaaaaaaaaaaaaaaaaaaaaaaaaaagcatatgactaaaaaaaaaaaaaaaaaaaaaaaaaaaaaaaaaaaaaaaaaaaaaaaaaaaaaaaaaaaaaaaaaaaaaa

SEQ ID NO: 53 - DNA, 2014 bp, synthetic construct
  source 1..2014: mol_type = other DNA; note; note (original language) = 5'UTR-Fluc-a 球蛋白3'UTR-120A (Mod.-120A)
gggaaataagagagaaaagaagagtaagaagaaatataagagccaccatggaagacgccaaaaacataaagaaaggcccggcgccattctatccgctggaagatggaaccgctggagagcaactgcataaggctatgaagagatacgccctggttcctggaacaattgcttttacagatgcacatatcgaggtggacatcacttacgctgagtacttcgaaatgtccgttcggttggcagaagctatgaaacgatatgggctgaatacaaatcacagaatcgtcgtatgcagtgaaaactctcttcaattctttatgccggtgttgggcgcgttatttatcggagttgcagttgcgcccgcgaacgacatttataatgaacgtgaattgctcaacagtatgggcatttcgcagcctaccgtggtgttcgtttccaaaaaggggttgcaaaaaattttgaacgtgcaaaaaaagctcccaatcatccaaaaaattattatcatggattctaaaacggattaccagggatttcagtcgatgtacacgttcgtcacatctcatctacctcccggttttaatgaatacgattttgtgccagagtccttcgatagggacaagacaattgcactgatcatgaactcctctggatctactggtctgcctaaaggtgtcgctctgcctcatagaactgcctgcgtgagattctcgcatgccagagatcctatttttggcaatcaaatcattccggatactgcgattttaagtgttgttccattccatcacggttttggaatgtttactacactcggatatttgatatgtggatttcgagtcgtcttaatgtatagatttgaagaagagctgtttctgaggagccttcaggattacaagattcaaagtgcgctgctggtgccaaccctattctccttcttcgccaaaagcactctgattgacaaatacgatttatctaatttacacgaaattgcttctggtggcgctcccctctctaaggaagtcggggaagcggttgccaagaggttccatctgccaggtatcaggcaaggatatgggctcactgagactacatcagctattctgattacacccgagggggatgataaaccgggcgcggtcggtaaagttgttccattttttgaagcgaaggttgtggatctggataccgggaaaacgctgggcgttaatcaaagaggcgaactgtgtgtgagaggtcctatgattatgtccggttatgtaaacaatccggaagcgaccaacgccttgattgacaaggatggatggctacattctggagacatagcttactgggacgaagacgaacacttcttcatcgttgaccgcctgaagtctctgattaagtacaaaggctatcaggtggctcccgctgaattggaatccatcttgctccaacaccccaacatcttcgacgcaggtgtcgcaggtcttcccgacgatgacgccggtgaacttcccgccgccgttgttgttttggagcacggaaagacgatgacggaaaaagagatcgtggattacgtcgccagtcaagtaacaaccgcgaaaaagttgcgcggaggagttgtgtttgtggacgaagtaccgaaaggtcttaccggaaaactcgacgcaagaaaaatcagagagatcctcataaaggccaagaagggcggaaagatcgccgtggattacaaggatgacgacgataagtaagggcccaccggttgataataggctggagcctcggtggccatgcttcttgccccttgggcctccccccagcccctcctccccttcctgcacccgtacccccgtggtctttgaataaagtctgagtgggcggcctcgagccgcggaaaaaaaaaaaaaaaaaaaaaaaaaaaaaaaaaaaaaaaaaaaaaaaaaaaaaaaaaaaaaaaaaaaaaaaaaaaaaaaaaaaaaaaaaaaaaaaaaaaaaaaaaaaaaaaaaaaaaaaattattgtttaaacatttaaattctaga

SEQ ID NO: 54 - DNA, 2004 bp, synthetic construct
  source 1..2004: mol_type = other DNA; note; note (original language) = 5'UTR-Fluc-a 球蛋白 3'UTR-A30L70 (Mod.-A30L70)
gggaaataagagagaaaagaagagtaagaagaaatataagagccaccatggaagacgccaaaaacataaagaaaggcccggcgccattctatccgctggaagatggaaccgctggagagcaactgcataaggctatgaagagatacgccctggttcctggaacaattgcttttacagatgcacatatcgaggtggacatcacttacgctgagtacttcgaaatgtccgttcggttggcagaagctatgaaacgatatgggctgaatacaaatcacagaatcgtcgtatgcagtgaaaactctcttcaattctttatgccggtgttgggcgcgttatttatcggagttgcagttgcgcccgcgaacgacatttataatgaacgtgaattgctcaacagtatgggcatttcgcagcctaccgtggtgttcgtttccaaaaaggggttgcaaaaaattttgaacgtgcaaaaaaagctcccaatcatccaaaaaattattatcatggattctaaaacggattaccagggatttcagtcgatgtacacgttcgtcacatctcatctacctcccggttttaatgaatacgattttgtgccagagtccttcgatagggacaagacaattgcactgatcatgaactcctctggatctactggtctgcctaaaggtgtcgctctgcctcatagaactgcctgcgtgagattctcgcatgccagagatcctatttttggcaatcaaatcattccggatactgcgattttaagtgttgttccattccatcacggttttggaatgtttactacactcggatatttgatatgtggatttcgagtcgtcttaatgtatagatttgaagaagagctgtttctgaggagccttcaggattacaagattcaaagtgcgctgctggtgccaaccctattctccttcttcgccaaaagcactctgattgacaaatacgatttatctaatttacacgaaattgcttctggtggcgctcccctctctaaggaagtcggggaagcggttgccaagaggttccatctgccaggtatcaggcaaggatatgggctcactgagactacatcagctattctgattacacccgagggggatgataaaccgggcgcggtcggtaaagttgttccattttttgaagcgaaggttgtggatctggataccgggaaaacgctgggcgttaatcaaagaggcgaactgtgtgtgagaggtcctatgattatgtccggttatgtaaacaatccggaagcgaccaacgccttgattgacaaggatggatggctacattctggagacatagcttactgggacgaagacgaacacttcttcatcgttgaccgcctgaagtctctgattaagtacaaaggctatcaggtggctcccgctgaattggaatccatcttgctccaacaccccaacatcttcgacgcaggtgtcgcaggtcttcccgacgatgacgccggtgaacttcccgccgccgttgttgttttggagcacggaaagacgatgacggaaaaagagatcgtggattacgtcgccagtcaagtaacaaccgcgaaaaagttgcgcggaggagttgtgtttgtggacgaagtaccgaaaggtcttaccggaaaactcgacgcaagaaaaatcagagagatcctcataaaggccaagaagggcggaaagatcgccgtggattacaaggatgacgacgataagtaagggcccaccggttgataataggctggagcctcggtggccatgcttcttgccccttgggcctccccccagcccctcctccccttcctgcacccgtacccccgtggtctttgaataaagtctgagtgggcggcctcgagccgcggaaaaaaaaaaaaaaaaaaaaaaaaaaaaaagcatatgactaaaaaaaaaaaaaaaaaaaaaaaaaaaaaaaaaaaaaaaaaaaaaaaaaaaaaaaaaaaaaaaaaaaaaattattgtttaaacatttaaattctaga

SEQ ID NO: 55 - DNA, 2206 bp, synthetic construct
  source 1..2206: mol_type = other DNA; note; note (original language) = a-1-球蛋白 5'UTR-Fluc- haplogroup U8b1b1 mitochondrion 3'UTR-A30L70 (BioN.)
agacgaactagtattcttctggtccccacagactcagagagaacccgccaccatggaagacgccaaaaacataaagaaaggcccggcgccattctatccgctggaagatggaaccgctggagagcaactgcataaggctatgaagagatacgccctggttcctggaacaattgcttttacagatgcacatatcgaggtggacatcacttacgctgagtacttcgaaatgtccgttcggttggcagaagctatgaaacgatatgggctgaatacaaatcacagaatcgtcgtatgcagtgaaaactctcttcaattctttatgccggtgttgggcgcgttatttatcggagttgcagttgcgcccgcgaacgacatttataatgaacgtgaattgctcaacagtatgggcatttcgcagcctaccgtggtgttcgtttccaaaaaggggttgcaaaaaattttgaacgtgcaaaaaaagctcccaatcatccaaaaaattattatcatggattctaaaacggattaccagggatttcagtcgatgtacacgttcgtcacatctcatctacctcccggttttaatgaatacgattttgtgccagagtccttcgatagggacaagacaattgcactgatcatgaactcctctggatctactggtctgcctaaaggtgtcgctctgcctcatagaactgcctgcgtgagattctcgcatgccagagatcctatttttggcaatcaaatcattccggatactgcgattttaagtgttgttccattccatcacggttttggaatgtttactacactcggatatttgatatgtggatttcgagtcgtcttaatgtatagatttgaagaagagctgtttctgaggagccttcaggattacaagattcaaagtgcgctgctggtgccaaccctattctccttcttcgccaaaagcactctgattgacaaatacgatttatctaatttacacgaaattgcttctggtggcgctcccctctctaaggaagtcggggaagcggttgccaagaggttccatctgccaggtatcaggcaaggatatgggctcactgagactacatcagctattctgattacacccgagggggatgataaaccgggcgcggtcggtaaagttgttccattttttgaagcgaaggttgtggatctggataccgggaaaacgctgggcgttaatcaaagaggcgaactgtgtgtgagaggtcctatgattatgtccggttatgtaaacaatccggaagcgaccaacgccttgattgacaaggatggatggctacattctggagacatagcttactgggacgaagacgaacacttcttcatcgttgaccgcctgaagtctctgattaagtacaaaggctatcaggtggctcccgctgaattggaatccatcttgctccaacaccccaacatcttcgacgcaggtgtcgcaggtcttcccgacgatgacgccggtgaacttcccgccgccgttgttgttttggagcacggaaagacgatgacggaaaaagagatcgtggattacgtcgccagtcaagtaacaaccgcgaaaaagttgcgcggaggagttgtgtttgtggacgaagtaccgaaaggtcttaccggaaaactcgacgcaagaaaaatcagagagatcctcataaaggccaagaagggcggaaagatcgccgtggattacaaggatgacgacgataagtaagggcccaccggctcgagctggtactgcatgcacgcaatgctagctgcccctttcccgtcctgggtaccccgagtctcccccgacctcgggtcccaggtatgctcccacctccacctgccccactcaccacctctgctagttccagacacctgctatactaatcgctagccgcgtcgctccccagggttggtcaatttcgtgccagccacaccgagacctggtccagagcccaagcacgccacacccccacgggaaacagcagtgattaacctttagcaataaacgaaagtttaactaacagcaatgcagctcaaaacgcttagcctagctcgagccgcggaaaaaaaaaaaaaaaaaaaaaaaaaaaaaagcatatgactaaaaaaaaaaaaaaaaaaaaaaaaaaaaaaaaaaaaaaaaaaaaaaaaaaaaaaaaaaaaaaaaaaaaaattattgtttaaacatttaaattctaga

SEQ ID NO: 56 - DNA, 2411 bp, synthetic construct
  source 1..2411: mol_type = other DNA; note = 5'UTR-Fluc- ACTG1 3'UTR-120A (B1)
gggaaataagagagaaaagaagagtaagaagaaatataagagccaccatggaagacgccaaaaacataaagaaaggcccggcgccattctatccgctggaagatggaaccgctggagagcaactgcataaggctatgaagagatacgccctggttcctggaacaattgcttttacagatgcacatatcgaggtggacatcacttacgctgagtacttcgaaatgtccgttcggttggcagaagctatgaaacgatatgggctgaatacaaatcacagaatcgtcgtatgcagtgaaaactctcttcaattctttatgccggtgttgggcgcgttatttatcggagttgcagttgcgcccgcgaacgacatttataatgaacgtgaattgctcaacagtatgggcatttcgcagcctaccgtggtgttcgtttccaaaaaggggttgcaaaaaattttgaacgtgcaaaaaaagctcccaatcatccaaaaaattattatcatggattctaaaacggattaccagggatttcagtcgatgtacacgttcgtcacatctcatctacctcccggttttaatgaatacgattttgtgccagagtccttcgatagggacaagacaattgcactgatcatgaactcctctggatctactggtctgcctaaaggtgtcgctctgcctcatagaactgcctgcgtgagattctcgcatgccagagatcctatttttggcaatcaaatcattccggatactgcgattttaagtgttgttccattccatcacggttttggaatgtttactacactcggatatttgatatgtggatttcgagtcgtcttaatgtatagatttgaagaagagctgtttctgaggagccttcaggattacaagattcaaagtgcgctgctggtgccaaccctattctccttcttcgccaaaagcactctgattgacaaatacgatttatctaatttacacgaaattgcttctggtggcgctcccctctctaaggaagtcggggaagcggttgccaagaggttccatctgccaggtatcaggcaaggatatgggctcactgagactacatcagctattctgattacacccgagggggatgataaaccgggcgcggtcggtaaagttgttccattttttgaagcgaaggttgtggatctggataccgggaaaacgctgggcgttaatcaaagaggcgaactgtgtgtgagaggtcctatgattatgtccggttatgtaaacaatccggaagcgaccaacgccttgattgacaaggatggatggctacattctggagacatagcttactgggacgaagacgaacacttcttcatcgttgaccgcctgaagtctctgattaagtacaaaggctatcaggtggctcccgctgaattggaatccatcttgctccaacaccccaacatcttcgacgcaggtgtcgcaggtcttcccgacgatgacgccggtgaacttcccgccgccgttgttgttttggagcacggaaagacgatgacggaaaaagagatcgtggattacgtcgccagtcaagtaacaaccgcgaaaaagttgcgcggaggagttgtgtttgtggacgaagtaccgaaaggtcttaccggaaaactcgacgcaagaaaaatcagagagatcctcataaaggccaagaagggcggaaagatcgccgtggattacaaggatgacgacgataagtaagggcccaccggccgactacctcatgaagatcctcactgagcgaggctacagcttcaccaccacggccgagcgggaaatcgtgcgcgacatcaaggagaagctgtgctacgtcgccctggacttcgagcaggagatggccaccgccgcatcctcctcttctctggagaagagctacgagctgcccgatggccaggtcatcaccattggcaatgagcggttccggtgtccggaggcgctgttccagccttccttcctgggtatggaatcttgcggcatccacgagaccaccttcaactccatcatgaagtgtgacgtggacatccgcaaagacctgtacgccaacacggtgctgtcgggcggcaccaccatgtacccgggcattgccgacaggatgcagaaggagatcaccgccctggcgcccagcaccatgaagatcaagatcatcgcacccccagagcgcaagtactcggtgtggatcggtggctccatcctggcctcactgtccaccttccagcagatgtggattagctcgagccgcggaaaaaaaaaaaaaaaaaaaaaaaaaaaaaaaaaaaaaaaaaaaaaaaaaaaaaaaaaaaaaaaaaaaaaaaaaaaaaaaaaaaaaaaaaaaaaaaaaaaaaaaaaaaaaaaaaaaaaaaattattgtttaaacatttaaattctaga

SEQ ID NO: 57 - DNA, 2027 bp, synthetic construct
  source 1..2027: mol_type = other DNA; note; note (original language) = ACTG1 5'UTR-Fluc-a 球蛋白 3'UTR-120A (A1)
ctctcgcactctgttcttccgccgctccgccgtcgcgtttctctgccggtcgcagccaccatggaagacgccaaaaacataaagaaaggcccggcgccattctatccgctggaagatggaaccgctggagagcaactgcataaggctatgaagagatacgccctggttcctggaacaattgcttttacagatgcacatatcgaggtggacatcacttacgctgagtacttcgaaatgtccgttcggttggcagaagctatgaaacgatatgggctgaatacaaatcacagaatcgtcgtatgcagtgaaaactctcttcaattctttatgccggtgttgggcgcgttatttatcggagttgcagttgcgcccgcgaacgacatttataatgaacgtgaattgctcaacagtatgggcatttcgcagcctaccgtggtgttcgtttccaaaaaggggttgcaaaaaattttgaacgtgcaaaaaaagctcccaatcatccaaaaaattattatcatggattctaaaacggattaccagggatttcagtcgatgtacacgttcgtcacatctcatctacctcccggttttaatgaatacgattttgtgccagagtccttcgatagggacaagacaattgcactgatcatgaactcctctggatctactggtctgcctaaaggtgtcgctctgcctcatagaactgcctgcgtgagattctcgcatgccagagatcctatttttggcaatcaaatcattccggatactgcgattttaagtgttgttccattccatcacggttttggaatgtttactacactcggatatttgatatgtggatttcgagtcgtcttaatgtatagatttgaagaagagctgtttctgaggagccttcaggattacaagattcaaagtgcgctgctggtgccaaccctattctccttcttcgccaaaagcactctgattgacaaatacgatttatctaatttacacgaaattgcttctggtggcgctcccctctctaaggaagtcggggaagcggttgccaagaggttccatctgccaggtatcaggcaaggatatgggctcactgagactacatcagctattctgattacacccgagggggatgataaaccgggcgcggtcggtaaagttgttccattttttgaagcgaaggttgtggatctggataccgggaaaacgctgggcgttaatcaaagaggcgaactgtgtgtgagaggtcctatgattatgtccggttatgtaaacaatccggaagcgaccaacgccttgattgacaaggatggatggctacattctggagacatagcttactgggacgaagacgaacacttcttcatcgttgaccgcctgaagtctctgattaagtacaaaggctatcaggtggctcccgctgaattggaatccatcttgctccaacaccccaacatcttcgacgcaggtgtcgcaggtcttcccgacgatgacgccggtgaacttcccgccgccgttgttgttttggagcacggaaagacgatgacggaaaaagagatcgtggattacgtcgccagtcaagtaacaaccgcgaaaaagttgcgcggaggagttgtgtttgtggacgaagtaccgaaaggtcttaccggaaaactcgacgcaagaaaaatcagagagatcctcataaaggccaagaagggcggaaagatcgccgtggattacaaggatgacgacgataagtaagggcccaccggttgataataggctggagcctcggtggccatgcttcttgccccttgggcctccccccagcccctcctccccttcctgcacccgtacccccgtggtctttgaataaagtctgagtgggcggcctcgagccgcggaaaaaaaaaaaaaaaaaaaaaaaaaaaaaaaaaaaaaaaaaaaaaaaaaaaaaaaaaaaaaaaaaaaaaaaaaaaaaaaaaaaaaaaaaaaaaaaaaaaaaaaaaaaaaaaaaaaaaaaattattgtttaaacatttaaattctaga

SEQ ID NO: 58 - RNA, 517 nt, synthetic construct
  source 1..517: mol_type = other RNA; note; note (original language) = B1 mRNA序列(ACTG1 3'UTR)
ccgactacctcatgaagatcctcactgagcgaggctacagcttcaccaccacggccgagcgggaaatcgtgcgcgacatcaaggagaagctgtgctacgtcgccctggacttcgagcaggagatggccaccgccgcatcctcctcttctctggagaagagctacgagctgcccgatggccaggtcatcaccattggcaatgagcggttccggtgtccggaggcgctgttccagccttccttcctgggtatggaatcttgcggcatccacgagaccaccttcaactccatcatgaagtgtgacgtggacatccgcaaagacctgtacgccaacacggtgctgtcgggcggcaccaccatgtacccgggcattgccgacaggatgcagaaggagatcaccgccctggcgcccagcaccatgaagatcaagatcatcgcacccccagagcgcaagtactcggtgtggatcggtggctccatcctggcctcactgtccaccttccagcagatgtggattag

SEQ ID NO: 59 - RNA, 282 nt, synthetic construct
  source 1..282: mol_type = other RNA; note; note (original language) = B2 mRNA序列(ATP6V0B)
atgatatgtgtgggtggggccgtgcctcacttttatttattgctggttttcctgggacagctggagctgtgtcccttagcctttcagaggcttggtgttcagggccctccctgcactcccctcttgctgcgtgttgatttggaggcactgcagtccaggccgagtcctcagtgcggggagcaggctgctgctgctgactctgtgcagctgcgcacctgtgtcccccacctccaccctcaacccatcttcctagtgtttgtgaaataaacttggtatttgtct

SEQ ID NO: 60 - RNA, 308 nt, synthetic construct
  source 1..308: mol_type = other RNA; note; note (original language) = B3 mRNA序列(ATP6V0B)
gttgaagaacttctctctaccgagcagcccgtaaccccctttttctccctcactgctgcaggagtctgctacaccatttttgatttgggcttccgctttgatgtggcatggttcctgacggagacttcgcccttcatgtggtccaacctgggcattggcctagctatctccctgtctgtggttggggcagcctggggcatctatattaccggctcctccatcattggtggaggagtgaaggcccccaggatcaagaccaagaacctggtcagcatcatcttctgtgaggctgtggccatctacggcat

SEQ ID NO: 61 - RNA, 226 nt, synthetic construct
  source 1..226: mol_type = other RNA; note; note (original language) = B4 mRNA序列(ATP6V0E1 3'UTR)
ggaagaagacatgctctacagtgctcagtctttgaggtgactatgcttgtgacctttcttatcagtatggtcaggcagtcagagtttgccttgactttttctcacattttatggccattttaacacgtggcaagggcaagctgctgaatgcaaacacgatctgaagagcagaaataaaattggaacttaagccttagcttacctaaatctcattaagattcttttt

SEQ ID NO: 62 - RNA, 461 nt, synthetic construct
  source 1..461: mol_type = other RNA; note; note (original language) = B5 mRNA序列(ATP6V0E1 3'UTR)
atgcaaaatcacctccaaaccagaccacttttcttgacttgcctgttttggccattagctgccttaaacgttaacagcacatttgaatgccttattctacaatgcagcgtgttttcctttgccttttttgcactttggtgaattacgtgcctccataacctgaactgtgccgactccacaaaacgattatgtactcttctgagatagaagatgctgttcttctgagagatacgttactctctccttggaatctgtggatttgaagatggctcctgccttctcacgtgggaatcagtgaagtgtttagaaactgctgcaagacaaacaagactccagtggggtggtcagtaggagagcacgttcagagggaagagccatctcaacagaatcgcaccaaactatactttcaggatgaatttcttctttctgccatcttttggaataaatattttcctcctttc

SEQ ID NO: 63 - RNA, 499 nt, synthetic construct
  source 1..499: mol_type = other RNA; note; note (original language) = B6 mRNA序列(CFL1 3'UTR)
gccccttctggccccctgcctggagcatctggcagccccacacctgcccttgggggttgcaggctgcccccttcctgccagaccggaggggctggggggatcccagcagggggagggcaatcccttcaccccagttgccaaacagaccccccaccccctggattttccttctccctccatcccttgacggttctggccttcccaaactgcttttgatcttttgattcctcttgggctgaagcagaccaagttccccccaggcaccccagttgtgggggagcctgtattttttttaacaacatccccattccccacctggtcctcccccttcccatgctgccaacttctaaccgcaatagtgactctgtgcttgtctgtttagttctgtgtataaatggaatgttgtggagatgacccctccctgtgccggctggttcctctcccttttcccctggtcacggctactcatggaagcaggaccagtaagggaccttcgatt

SEQ ID NO: 64 - RNA, 282 nt, synthetic construct
  source 1..282: mol_type = other RNA; note; note (original language) = B7 mRNA序列 (CFL1 3'UTR)
gccccttctggccccctgcctggagcatctggcagccccacacctgcccttgggggttgcaggctgcccccttcctgccagaccggaggggctggggggatcccagcagggggagggcaatcccttcaccccagttgccaaacagaccccccaccccctggattttccttctccctccatcccttgacggttctggccttcccaaactgcttttgatcttttgattcctcttgggctgaagcagaccaagttccccccaggcaccccagttgtgggggagcc

SEQ ID NO: 65 - RNA, 361 nt, synthetic construct
  source 1..361: mol_type = other RNA; note; note (original language) = B8 mRNA序列 (CFL1 3'UTR)
gccccttctggccccctgcctggagcatctggcagccccacacctgcccttgggggttgcaggctgcccccttcctgccagaccggaggggctggggggatcccagcagggggagggcaatcccttcaccccagttgccaaacagaccccccaccccctggattttccttctccctccatcccttgacggttctggccttcccaaactgcttttgatcttttgattcctcttgggctgaagcagaccaagttccccccaggcaccccagttgtgggggagcctgtattttttttaacaacatccccattccccacctggtcctcccccttcccatgctgccaacttctaaccgcaatagtg

SEQ ID NO: 66 - RNA, 128 nt, synthetic construct
  source 1..128: mol_type = other RNA; note; note (original language) = B9 mRNA序列 (COX4I1 3'UTR)
gagatgctggcctgcgcctgcacctgcgcctggctctgtcaccgccatgcaactccatgcctatttactggaaacctgttatgccaaacagttgtaccactgctaataaatgaccagtttacctgaaa

SEQ ID NO: 67 - RNA, 319 nt, synthetic construct
  source 1..319: mol_type = other RNA; note; note (original language) = B10 mRNA序列 (COX4I1 3'UTR)
agggacccacaggcgcgcccagcagctctcggaagcgttgtatcgcattaagttcaaggagagctttgctgagatgaacaggggctcgaacgagtggaagacggttgtgggcggtgccatgttcttcatcggtttcaccgcgctcgttatcatgtggcagaagcactatgggcttagcctccaagtgggactacgaaaagaacgagtggaagaagtgagagatgctggcctgcgcctgcacctgcgcctggctctgtcaccgccatgcaactccatgcctatttactggaaacctgttatgccaaacagttgtaccact

SEQ ID NO: 68 - RNA, 303 nt, synthetic construct
  source 1..303: mol_type = other RNA; note; note (original language) = B11 mRNA序列 (COX4I1 3'UTR)
agaggaccttctgcttttagcttattttgttgctaactttttacaaacaaagggctaattttaaaatgtcagtgttgtcagtggtcagaaaccgtgtgtttgagcgggtgttgagtggcaggtggctctgctgacctggtggctggtgtgtcgggaggatttaacctgtgtgagggattggcctagaaacaacctgttgagatagtcttgccccataacctgtctcacaccgtagtgtacggccccctcccgcaaagctttgacaaagagtgggtggccaagcagaccaagaggatgctggac

SEQ ID NO: 69 - RNA, 232 nt, synthetic construct
  source 1..232: mol_type = other RNA; note; note (original language) = B12 mRNA序列 (CTSB 3'UTR)
tctgccgtgggcctgtcgtgccagtcctgggggcgagatcgggagaatcacgtcctggaactgcatgttcttgcgactcttgggacttcatcttaacttctcgctgccccagccatgttttcaaccatggcatccctcccccaattagttccctgtcatcctcgtcaaccttctctgtaagtgcctggtaagcttgcccttgcttaagaactcaaaacatagctgtgctcta

SEQ ID NO: 70 - RNA, 115 nt, synthetic construct
  source 1..115: mol_type = other RNA; note; note (original language) = B13 mRNA序列 (FAM166A 3'UTR)
aaatgctttaatggtggtgtctgtacagcatggatgtggacagggaaaacagcaagtgcacacagtgggacaggccacaggacaggctgggagtgaataaagagttcacactgct

SEQ ID NO: 71 - RNA, 196 nt, synthetic construct
  source 1..196: mol_type = other RNA; note; note (original language) = B14 mRNA序列 (NDUFB9 3'UTR)
tatctaagtgtatcaatttaacatttataatcaccttacaagtaagttaaagtgcattccctggtcgttttggctttgtctttgattttgcttcagatctccttctctttagtcctttgtctgacttttttgccttcttgctatactttccctcaacctgcctctccactattttcttaggcatttttcagtcatg

SEQ ID NO: 72 - RNA, 54 nt, synthetic construct
  source 1..54: mol_type = other RNA; note; note (original language) = A1 mRNA序列 (ACTG1 5'UTR)
ctctcgcactctgttcttccgccgctccgccgtcgcgtttctctgccggtcgca

SEQ ID NO: 73 - RNA, 185 nt, synthetic construct
  source 1..185: mol_type = other RNA; note; note (original language) = A2 mRNA序列 (ATP6V0B 5'UTR)
gggcgggcggacagactgcgggacggacggtggacgctgggacgcgtttgtagctccggccccgccgttccgacccccgccgccgtcgccgccatgacggggctagcactgctctactccggggtcttcgtggccttctgggcctgcgcgctggccgtgggttcctgacggagacttcgcccttc

SEQ ID NO: 74 - RNA, 81 nt, synthetic construct
  source 1..81: mol_type = other RNA; note; note (original language) = A3 mRNA序列 (ATP6V0B 5'UTR)
agactgcgggacggacggtggacgctgggacgcgtttgtagctccggccccgccgttccgacccccgccgccgtcgccgcc

SEQ ID NO: 75 - RNA, 30 nt, synthetic construct
  source 1..30: mol_type = other RNA; note; note (original language) = A4 mRNA序列 (ATP6V0E1 5'UTR)
ggggtaggggttggcgctcaggcggcgacc

SEQ ID NO: 76 - RNA, 80 nt, synthetic construct
  source 1..80: mol_type = other RNA; note; note (original language) = A5 mRNA序列 (ATP6V0E1 5'UTR)
gtcacgcggtcagctattgacacttcctggtgggatccgagtgaggcgacggggtaggggttggcgctcaggcggcgacc

SEQ ID NO: 77 - RNA, 234 nt, synthetic construct
  source 1..234: mol_type = other RNA; note; note (original language) = A6 mRNA序列 (CFL1 5'UTR)
ggccggcgggaagactccgttacccagcgagcgaggcggcggcgcagggccagcggactccatttcccgtcggctcgcggtgggagcgccggaagcccgccccacccctcattgtgcggctcctactaaacggaaggggccgggagaggccgcgttcagtcgggtcccggcagcggctgcagcgctctcgtcttctgcggctctcggtgccctctccttttcgtttccggaaac

SEQ ID NO: 78 - RNA, 128 nt, synthetic construct
  source 1..128: mol_type = other RNA; note; note (original language) = A7 mRNA序列 (CFL1 5'UTR)
ctcctggctcgggcaccccgaagcacgacgcagagtaggaagagtttaaagacctcgaggcctctgggcacttgagtttggcctccggtgtggctgtctctgatggtgtcatcaaggtgttcaacgac

SEQ ID NO: 79 - RNA, 151 nt, synthetic construct
  source 1..151: mol_type = other RNA; note; note (original language) = A8 mRNA序列 (CFL1 5'UTR)
acgtggccggcttcttctgcagttccggggagtttgggggaccagatttaccttggattgcccctccctctcctggctcgggcaccccgaagcacgacgcagagcctccggtgtggctgtctctgatggtgtcatcaaggtgttcaacgac

SEQ ID NO: 80 - RNA, 70 nt, synthetic construct
  source 1..70: mol_type = other RNA; note; note (original language) = A9 mRNA序列 (COX4I1 5'UTR)
gcggccttgctctcttccggtcgcgggacaccgggtgtagagggcggtcgcggcgggcagtggcggcaga

SEQ ID NO: 81 - RNA, 46 nt, synthetic construct
  source 1..46: mol_type = other RNA; note; note (original language) = A10 mRNA序列 (COX4I1 5'UTR)
gggacaccgggtgtagagggcggtcgcggcgggcagtggcggcaga

SEQ ID NO: 82 - RNA, 71 nt, synthetic construct
  source 1..71: mol_type = other RNA; note; note (original language) = A11 mRNA序列 (COX4I1 5'UTR)
cgcggccttgctctcttccggtcgcgggacaccgggtgtagagggcggtcgcggcgggcagtggcggcaga

SEQ ID NO: 83 - RNA, 137 nt, synthetic construct
  source 1..137: mol_type = other RNA; note; note (original language) = A12 mRNA序列 (CUSB 5'UTR)
ggccggggctggcccaggctacggcggctgcagggctccggcaaccgctccggcaacgccaaccgctccgctgcgcgcaggctgggctgcaggctctcggctgcagcgctgggtggatctaggatccggcttccaac

SEQ ID NO: 84 - RNA, 55 nt, synthetic construct
  source 1..55: mol_type = other RNA; note; note (original language) = A13 mRNA序列 (FAM166A 5'UTR)
aagggagctggatgccgggagggactggagccagcaaggccagagtgaaagcaaa

SEQ ID NO: 85 - RNA, 56 nt, synthetic construct
  source 1..56: mol_type = other RNA; note; note (original language) = A14 mRNA序列 (NDUFB9 5'UTR)
gcagcaggcgtgcagtttcccggctctccgcgcggccggggaaggtcagcgccgta

SEQ ID NO: 86 - RNA, 68 nt, synthetic construct
  source 1..68: mol_type = other RNA; note; note (original language) = A15 mRNA序列 (CHCHD10 5'UTR)
ggcatttgtccccgcgacagcaccgctgccgccgtctctaaggtcgcccgggtcccaccgccgccacc

SEQ ID NO: 87 - RNA, 46 nt, synthetic construct
  source 1..46: mol_type = other RNA; note; note (original language) = A16 mRNA序列 (CHCHD10 5'UTR)
ccgctgccgccgtctctaaggtcgcccgggtcccaccgccgccacc

SEQ ID NO: 88 - RNA, 41 nt, synthetic construct
  source 1..41: mol_type = other RNA; note; note (original language) = A17 mRNA序列 (SLC38A2 5'UTR)
atgtcttttttgtgtgtttgttttcatggtattcctatgaa

SEQ ID NO: 89 - RNA, 48 nt, synthetic construct
  source 1..48: mol_type = other RNA; note; note (original language) = A18 mRNA序列 (NDUFA11 5'UTR)
gcttcccgagctggcggggtccgtggtgcgggatcgagattgcgggct

SEQ ID NO: 90 - RNA, 69 nt, synthetic construct
  source 1..69: mol_type = other RNA; note; note (original language) = A19 mRNA序列 (NDUFV3 5'UTR)
ggcggctgttcaggcgcgggtgcgcgcgcagctgctgtggccctgcttggtgcgcccgctgtcaccgcc

SEQ ID NO: 91 - RNA, 128 nt, synthetic construct
  source 1..128: mol_type = other RNA; note; note (original language) = A20 mRNA序列 (PRDX5 5'UTR)
cgcgcctgcgcagtggaggcggcccaggcccgccttccgcagggtgtcgccgctgtgccgctagcggtgccccgcctgctgcggtggcaccagccaggaggcggagtggaagtggccgtggggcgggt

SEQ ID NO: 92 - RNA, 59 nt, synthetic construct
  source 1..59: mol_type = other RNA; note; note (original language) = A21 mRNA序列 (GUK1 5'UTR)
cagcagatggggactagaggccgcactgctatccacagcctctcttctcacccccaggc

SEQ ID NO: 93 - RNA, 68 nt, synthetic construct
  source 1..68: mol_type = other RNA; note; note (original language) = A22 mRNA序列 (GUK1 5'UTR)
gctggccgggctggctgcggccgccctgggccgggccccaccggacgcctctcttctcacccccaggc

SEQ ID NO: 94 - RNA, 96 nt, synthetic construct
  source 1..96: mol_type = other RNA; note; note (original language) = A23 mRNA序列 (GUK1 5'UTR)
agaggtggccccggatgctgcggcgcccgctggccgggctggctgcggccgccctgggccgggccccaccggacgcctctcttctcacccccaggc

SEQ ID NO: 95 - RNA, 37 nt, synthetic construct
  source 1..37: mol_type = other RNA; note; note (original language) = A24 mRNA序列 (IAH1 5'UTR)
tggctggcggccccgccccgccccgcccggctgctcc

SEQ ID NO: 96 - RNA, 59 nt, synthetic construct
  source 1..59: mol_type = other RNA; note; note (original language) = A25 mRNA序列 (ABHD16A 5'UTR)
ggagggcggggccggcagggggacctgctgctggaagagcagcggcccgagccggggcc

SEQ ID NO: 97 - RNA, 132 nt, synthetic construct
  source 1..132: mol_type = other RNA; note; note (original language) = A26 mRNA序列 (SLC25A39 5'UTR)
tttcggcgtcggcctaggtgcgctgcgagcgcgcgcggaccgcgcacaggcggcggagccggtatgggcccgcctgaccctgggcgccgcgccgcacgagcaccagcctagagccaggactgaagcttcaag

SEQ ID NO: 98 - RNA, 51 nt, synthetic construct
  source 1..51: mol_type = other RNA; note; note (original language) = A27 mRNA序列 (AUPIF1 5'UTR)
cgagagactgcttgctgcggcagagacgccagaggtgcagctccagcagca

SEQ ID NO: 99 - RNA, 71 nt, synthetic construct
  source 1..71: mol_type = other RNA; note; note (original language) = A28 mRNA序列 (ANAPC11 5'UTR)
cggagtttcgtcatgttggccaggcccatttgagatctttgaagatatcctcaacgtgaggctctgctgcc

SEQ ID NO: 100 - RNA, 55 nt, synthetic construct
  source 1..55: mol_type = other RNA; note; note (original language) = A29 mRNA序列 (ANAPC11 5'UTR)
gggcgcggcttcggcgggcggcagccgctgcagacgagctgcgggctctgctgcc

SEQ ID NO: 101 - RNA, 48 nt, synthetic construct
  source 1..48: mol_type = other RNA; note; note (original language) = A30 mRNA序列 (CCDC12 5'UTR)
gcctgcgcgatgcaagacgggagaaaaggaggggcgtacgcgggcaag

SEQ ID NO: 102 - RNA, 132 nt, synthetic construct
  source 1..132: mol_type = other RNA; note; note (original language) = A31 mRNA序列 (MRPL14 5'UTR)
atcgcgtccgccgggctgggcctggcgcgcaggcgctaggaagaggccgcgtggggcgaaggcggcgcttggctggtggggcccgcggcgggattttcccgggcggcgagagcggatctatcttgggatccc

SEQ ID NO: 103 - RNA, 27 nt, synthetic construct
  source 1..27: mol_type = other RNA; note; note (original language) = A32 mRNA序列 (APOA1BP 5'UTR)
gccgggggcgcgcgctctgcgagctgg

SEQ ID NO: 104 - RNA, 43 nt, synthetic construct
  source 1..43: mol_type = other RNA; note; note (original language) = A33 mRNA序列 (APOA1BP 5'UTR)
gccggggccgggccgggccgggggcgcgcgctctgcgagctgg

SEQ ID NO: 105 - RNA, 47 nt, synthetic construct
  source 1..47: mol_type = other RNA; note; note (original language) = Mod. 5'UTR mRNA序列
gggaaataagagagaaaagaagagtaagaagaaatataagagccacc

SEQ ID NO: 106 - RNA, 119 nt, synthetic construct
  source 1..119: mol_type = other RNA; note; note (original language) = a-球蛋白 3'UTR mRNA序列
tgataataggctggagcctcggtggccatgcttcttgccccttgggcctccccccagcccctcctccccttcctgcacccgtacccccgtggtctttgaataaagtctgagtgggcggc

SEQ ID NO: 107 - RNA, 52 nt, synthetic construct; identical to SEQ ID NO: 50
  source 1..52: mol_type = other RNA; note; note (original language) = a-1 球蛋白 5'UTR mRNA序列

SEQ ID NO: 108 - RNA, 317 nt, synthetic construct
  source 1..317: mol_type = other RNA; note; note (original language) = haplogroup U8b1b1 mitochondrion 3'UTR mRNA序列
ctcgagctggtactgcatgcacgcaatgctagctgcccctttcccgtcctgggtaccccgagtctcccccgacctcgggtcccaggtatgctcccacctccacctgccccactcaccacctctgctagttccagacacctgctatactaatcgctagccgcgtcgctccccagggttggtcaatttcgtgccagccacaccgagacctggtccagagcccaagcacgccacacccccacgggaaacagcagtgattaacctttagcaataaacgaaagtttaactaacagcaatgcagctcaaaacgcttagcctag

SEQ ID NO: 109 - protein, 728 aa, Homo sapiens
  source 1..728: note; note (original language) = hHGF氨基酸序列
MWVTKLLPALLLQHVLLHLLLLPIAIPYAEGQRKRRNTIHEFKKSAKTTLIKIDPALKIKTKKVNTADQCANRCTRNKGLPFTCKAFVFDKARKQCLWFPFNSMSSGVKKEFGHEFDLYENKDYIRNCIIGKGRSYKGTVSITKSGIKCQPWSSMIPHEHSFLPSSYRGKDLQENYCRNPRGEEGGPWCFTSNPEVRYEVCDIPQCSEVECMTCNGESYRGLMDHTESGKICQRWDHQTPHRHKFLPERYPDKGFDDNYCRNPDGQPRPWCYTLDPHTRWEYCAIKTCADNTMNDTDVPLETTECIQGQGEGYRGTVNTIWNGIPCQRWDSQYPHEHDMTPENFKCKDLRENYCRNPDGSESPWCFTTDPNIRVGYCSQIPNCDMSHGQDCYRGNGKNYMGNLSQTRSGLTCSMWDKNMEDLHRHIFWEPDASKLNENYCRNPDDDAHGPWCYTGNPLIPWDYCPISRCEGDTTPTIVNLDHPVISCAKTKQLRVVNGIPTRTNIGWMVSLRYRNKHICGGSLIKESWVLTARQCFPSRDLKDYEAWLGIHDVHGRGDEKCKQVLNVSQLVYGPEGSDLVLMKLARPAVLDDFVSTIDLPNYGCTIPEKTSCSVYGWGYTGLINYDGLLRVAHLYIMGNEKCSQHHRGKVTLNESEICAGAEKIGSGPCEGDYGGPLVCEQHKMRMVLGVIVPGRGCAIPNRPGIFVRVAYYAKWIHKIILTYKVPQS

SEQ ID NO: 110 - DNA, 2187 bp, synthetic construct
  source 1..2187: mol_type = other DNA; note; note (original language) = hHGF核苷酸序列
atgtgggtgaccaaactcctgccagccctgctgctgcagcatgtcctcctgcatctcctcctgctccccatcgccatcccctatgcagagggacaaaggaaaagaagaaatacaattcatgaattcaaaaaatcagcaaagactaccctaatcaaaatagatccagcactgaagataaaaaccaaaaaagtgaatactgcagaccaatgtgctaatagatgtactaggaataaaggacttccattcacttgcaaggcttttgtttttgataaagcaagaaaacaatgcctctggttccccttcaatagcatgtcaagtggagtgaaaaaagaatttggccatgaatttgacctctatgaaaacaaagactacattagaaactgcatcattggtaaaggacgcagctacaagggaacagtatctatcactaagagtggcatcaaatgtcagccctggagttccatgataccacacgaacacagctttttgccttcgagctatcggggtaaagacctacaggaaaactactgtcgaaatcctcgaggggaagaagggggaccctggtgtttcacaagcaatccagaggtacgctacgaagtctgtgacattcctcagtgttcagaagttgaatgcatgacctgcaatggggagagttatcgaggtctcatggatcatacagaatcaggcaagatttgtcagcgctgggatcatcagacaccacaccggcacaaattcttgcctgaaagatatcccgacaagggctttgatgataattattgccgcaatcccgatggccagccgaggccatggtgctatactcttgaccctcacacccgctgggagtactgtgcaattaaaacatgcgctgacaatactatgaatgacactgatgttcctttggaaacaactgaatgcatccaaggtcaaggagaaggctacaggggcactgtcaataccatttggaatggaattccatgtcagcgttgggattctcagtatcctcacgagcatgacatgactcctgaaaatttcaagtgcaaggacctacgagaaaattactgccgaaatccagatgggtctgaatcaccctggtgttttaccactgatccaaacatccgagttggctactgctcccaaattccaaactgtgatatgtcacatggacaagattgttatcgtgggaatggcaaaaattatatgggcaacttatcccaaacaagatctggactaacatgttcaatgtgggacaagaacatggaagacttacatcgtcatatcttctgggaaccagatgcaagtaagctgaatgagaattactgccgaaatccagatgatgatgctcatggaccctggtgctacacgggaaatccactcattccttgggattattgccctatttctcgttgtgaaggtgataccacacctacaatagtcaatttagaccatcccgtaatatcttgtgccaaaacgaaacaattgcgagttgtaaatgggattccaacacgaacaaacataggatggatggttagtttgagatacagaaataaacatatctgcggaggatcattgataaaggagagttgggttcttactgcacgacagtgtttcccttctcgagacttgaaagattatgaagcttggcttggaattcatgatgtccacggaagaggagatgagaaatgcaaacaggttctcaatgtttcccagctggtatatggccctgaaggatcagatctggttttaatgaagcttgccaggcctgctgtcctggatgattttgttagtacgattgatttacctaattatggatgcacaattcctgaaaagaccagttgcagtgtttatggctggggctacactggattgatcaactatgatggcctattacgagtggcacatctctatataatgggaaatgagaaatgcagccagcatcatcgagggaaggtgactctgaatgagtctgaaatatgtgctggggctgaaaagattggatcaggaccatgtgagggggattatggtggcccacttgtttgtgagcaacataaaatgagaatggttcttggtgtcattgttcctggtcgtggatgtgccattccaaatcgtcctggtatttttgtccgagtagcatattatgcaaaatggatacacaaaattattttaacatataaggtaccacagtcatag

SEQ ID NO: 111 - DNA, 2187 bp, synthetic construct
  source 1..2187: mol_type = other DNA; note; note (original language) = hHGF密码子优化序列1(hHGF-OS1)
atgtgggtgaccaaactgctccccgctctgctgctgcagcatgtgctgctccacctgctgctgctgccaatcgccatcccctacgctgaaggacagcggaagcgcagaaacacaattcacgaattcaagaagtccgccaaaacaacactgatcaagatcgaccctgccctgaaaatcaaaaccaagaaggtgaacactgccgatcagtgcgccaacagatgcacaagaaacaaaggcctgcccttcacatgcaaggcctttgtgttcgacaaggccagaaagcagtgcctgtggttccctttcaacagcatgagctctggcgtgaagaaagagttcggccacgaattcgacctgtacgagaacaaggattacatcagaaattgtatcatcggcaagggcagaagctacaaaggcacagtgtccatcaccaaaagcggcattaagtgtcagccttggagcagcatgatccctcacgagcacagcttcctgcctagctcttacagaggcaaggacctgcaggagaattactgccggaaccctagaggcgaggaaggcggcccttggtgctttaccagcaaccctgaggtgcggtacgaggtgtgtgacatcccccagtgcagcgaagtggaatgcatgacctgtaatggcgagagctacagaggcctcatggaccatacagagagcggaaagatttgtcaaagatgggatcaccagacacctcacagacacaaattcctgcccgaaagatatcctgacaagggcttcgacgacaactactgcagaaatcctgatggccaacccagaccttggtgctacaccctggatcctcataccagatgggagtactgtgccatcaagacctgcgctgataataccatgaacgacaccgatgtgcctctggaaacaaccgagtgcatccagggacagggcgaaggctaccggggcaccgtgaacaccatctggaacggcatcccctgccagagatgggacagccagtacccccacgaacacgatatgacccctgagaacttcaagtgcaaggacctgagagaaaattactgcagaaacccagacggaagcgagtctccttggtgttttaccaccgaccccaacatccgggtgggttactgcagccaaatccccaattgcgacatgagccacggccaggactgctaccggggaaacggcaaaaactacatgggcaatctgagccagacccggagcggtctgacctgctccatgtgggataagaacatggaagatctgcaccggcacatcttctgggagcctgacgcttctaagctgaacgagaactactgtaggaacccagacgacgatgcccacggtccctggtgctacaccggcaacccgctgatcccttgggactattgtcctatcagccgctgcgagggcgatacaacacctaccatcgtgaacctggaccaccctgtgatctcttgcgccaagaccaagcagctgagagtggtgaacggcatcccaacacggaccaacatcggatggatggtctccctgagataccggaacaagcacatctgcggcggctctctgatcaaggaatcttgggtcctgaccgccagacagtgcttccccagccgggacctgaaggactatgaggcctggctgggaatccacgacgtgcacggcagaggcgacgagaagtgcaagcaagtgctgaacgtgtcccagctggtgtacggccctgagggatctgatctggtcctgatgaaactggccagacccgccgtgctggacgactttgtgtccaccatcgacctgcctaactacggctgcaccatccctgaaaagaccagctgcagcgtgtacggctggggctatacaggcctgatcaactacgacggtctgctgcgggttgctcacctgtacatcatgggcaacgagaagtgcagccagcaccacagaggaaaggttacacttaacgagagcgagatctgcgccggcgccgagaaaatcggctccggcccttgtgaaggcgactacggaggccctctggtgtgcgaacagcacaagatgagaatggtgctgggcgtgatcgtgcccggaagaggctgtgcaatccctaataggcccggcattttcgtgcgggtggcctactacgccaagtggatccacaagatcatcctgacgtacaaggtgcctcagagctga

SEQ ID NO: 112 - DNA, 2187 bp, synthetic construct
  source 1..2187: mol_type = other DNA; note; note (original language) = hHGF密码子优化序列2(hHGF-OS2)
atgtgggtcaccaaactgctgcccgccctgctgctgcagcacgtgctcctgcacctgctgctgctgcctatcgccatcccttacgccgaaggccagagaaagcggagaaataccattcacgaatttaagaagagcgccaagaccacactgatcaagatcgaccctgccctgaaaatcaagaccaagaaagtgaacacagccgaccaatgcgctaatagatgcacaagaaacaaaggcctgcctttcacctgcaaggccttcgtgttcgataaggccagaaagcagtgcctgtggttccccttcaacagcatgagcagcggcgtgaagaaagaattcggtcacgagttcgacctgtacgagaataaggactacattagaaactgcatcatcggcaagggccggagctacaagggcaccgtgagcatcaccaagtctggcatcaagtgccagccatggagttccatgatccctcatgagcacagcttcctgccaagctcttaccggggaaaggatctgcaggagaactattgtagaaatcccagaggcgaggaaggaggaccctggtgttttaccagcaacccagaggtgcggtacgaggtgtgcgacataccccagtgcagcgaggtggaatgcatgacatgcaacggcgagagctaccggggcctgatggaccacacagagagcggcaaaatctgccaaagatgggatcaccagacccctcataggcacaagttcctgcccgagagataccctgacaagggcttcgacgacaattactgccggaaccctgatggacagcctagaccttggtgctacaccctggaccctcacaccagatgggaatactgcgccatcaagacatgtgccgataacaccatgaacgacaccgatgtgccactcgagacaactgagtgtatccagggccagggcgagggctacaggggcaccgtgaacaccatctggaacggcatcccttgtcagcggtgggacagccaatacccccacgaacatgatatgaccccagaaaacttcaagtgcaaagatctgcgggaaaactactgtagaaaccctgacggctccgagagcccttggtgcttcaccaccgaccctaacatcagggtgggctactgtagccagatccccaactgcgacatgagccacggtcaggactgctacagaggaaacggcaagaattacatgggcaacctgagccagaccagaagcggcctgacctgcagcatgtgggacaaaaacatggaagatctgcaccggcacatcttttgggagcctgacgccagcaagctgaatgagaactactgtcggaaccctgacgacgatgctcacggcccttggtgctacacaggcaaccctctgatcccttgggactattgtcctattagcaggtgtgaaggcgacacgacccctacaatcgtgaacctggatcacccagtgatcagctgtgctaaaacaaagcaactgagagtggtgaatggtatcccgacccggaccaacatcggatggatggtcagcctgcggtacagaaacaagcacatctgcggcggtagcctgatcaaggaatcctgggtgttgacagccagacagtgttttcccagcagagatctgaaggactacgaggcctggctgggcatccacgacgtgcacggcagaggcgacgagaagtgcaagcaggttctgaacgtgtcccagctggtgtacggccccgagggctctgatctggttctgatgaagcttgctagacccgctgtgctggatgacttcgtgtccaccatcgacctgccaaattacggatgtacaattcctgaaaagacctcctgttctgtgtacggctggggctacaccggactcatcaactatgacggcctgctgagagtggcccacctgtatatcatgggcaacgagaagtgcagccagcaccatagaggcaaggtgaccctgaacgagtctgaaatctgcgccggagccgagaaaatcggatctggcccctgcgaaggagattacggcggccctctggtctgcgagcagcacaagatgagaatggtgctgggcgtgatcgtgcccggcagaggctgcgccatccctaaccggcctggaatcttcgtgcgcgtggcctattacgccaaatggatccacaaaatcatcctgacatacaaggtcccacagtcttga

SEQ ID NO: 113 - DNA, 2187 bp, synthetic construct
  source 1..2187: mol_type = other DNA; note; note (original language) = hHGF密码子优化序列3(hHGF-OS3)
atgtgggtgaccaagctgctgcccgccctgctcctgcagcacgtgctgctgcacctgctcctgctgcccatcgccatcccctacgccgaggggcagagaaagagaagaaacaccatccacgagttcaagaagagcgccaagaccaccctgatcaagatcgaccccgccctgaagatcaagaccaagaaggtgaacaccgccgatcagtgcgccaacagatgcacaagaaacaagggcctgcccttcacctgcaaggccttcgtgttcgacaaggctagaaagcagtgcctgtggttccccttcaacagcatgagcagcggcgtgaagaaggagttcggccacgagttcgacctgtacgagaacaaggactacatcagaaactgcatcatcggcaagggcagaagctacaagggcaccgtgagcatcaccaagagcggcatcaagtgtcagccctggagcagcatgatcccccatgagcacagcttcctgcctagcagctacagagggaaggacctgcaagagaactactgcagaaaccctagaggcgaggagggcggcccttggtgtttcacaagcaatcccgaggtgagatacgaggtgtgcgacatccctcagtgcagcgaggtggagtgcatgacctgcaacggcgaaagctatagaggcctgatggaccacaccgagagcggcaagatttgtcagcggtgggatcaccaaaccccccacagacacaagttcctgcccgagagataccccgacaagggcttcgacgacaattactgtagaaaccccgacgggcagcctagaccctggtgttacaccctggacccccacacaagatgggagtactgcgccatcaagacctgcgccgacaacaccatgaacgacaccgacgtgcccctggagaccaccgagtgcatccaaggccaaggcgagggctacagaggcaccgtgaacaccatctggaacggcattccctgtcagagatgggacagccaatacccccatgaacacgatatgacccccgagaacttcaagtgcaaggacctgagagagaactactgccggaaccccgatggcagcgaatccccttggtgcttcaccaccgaccccaacatcagagtgggctactgcagccaaatccccaactgcgacatgagccacggccaagactgttacagagggaacggcaagaactacatgggcaacctgagccaaacaagaagcggcctgacctgcagcatgtgggacaagaacatggaggacctgcacagacacatcttctgggagcccgacgctagcaagctgaacgagaactactgtcggaaccccgacgacgatgcccacggcccctggtgctacaccggcaaccccctgatcccctgggactactgccccatcagcagatgcgagggcgacaccacccccaccatcgtgaacctggaccaccccgtgatcagctgtgccaagaccaagcaactgagagtggtgaacggcatccccacaagaaccaacattggctggatggtgagcctgagatacagaaacaagcacatctgcggcggcagcctgatcaaggagagctgggtgctgaccgctagacagtgcttccctagcagagacctgaaggactacgaggcctggctgggcatccacgacgtgcacggcagaggcgacgagaagtgtaaacaagtgctgaacgtgagccaactggtgtacggccccgagggcagcgacctggtgctgatgaagctggctagacccgccgtgctggacgacttcgtgagcaccatcgacctgcccaactacggctgcaccatccccgagaagacaagctgcagcgtgtacggctggggctacaccggcctgatcaactacgacggcctgctgagagtggcccacctgtacatcatgggcaacgagaagtgcagccaacaccaccggggcaaagtgaccctgaacgagagcgagatctgcgccggggctgagaaaatcggcagcggcccctgcgagggggactacgggggccccctggtgtgcgagcagcacaagatgagaatggtgctgggcgtgatcgtgcccggcagaggctgcgccatccccaacagacccggcatcttcgtgagagtggcctactacgccaagtggatccacaagatcatcctgacctacaaggtgcctcagagctga

SEQ ID NO: 114 - DNA, 2512 bp, synthetic construct
  source 1..2512: mol_type = other DNA; note; note (original language) = 5'UTR-hHGF-α 球蛋白 3'UTR-A30L70 (Mod.-hHGF-OS2)
gggaaataagagagaaaagaagagtaagaagaaatataagagccaccgctagccttaaggccaccatgtgggtcaccaaactgctgcccgccctgctgctgcagcacgtgctcctgcacctgctgctgctgcctatcgccatcccttacgccgaaggccagagaaagcggagaaataccattcacgaatttaagaagagcgccaagaccacactgatcaagatcgaccctgccctgaaaatcaagaccaagaaagtgaacacagccgaccaatgcgctaatagatgcacaagaaacaaaggcctgcctttcacctgcaaggccttcgtgttcgataaggccagaaagcagtgcctgtggttccccttcaacagcatgagcagcggcgtgaagaaagaattcggtcacgagttcgacctgtacgagaataaggactacattagaaactgcatcatcggcaagggccggagctacaagggcaccgtgagcatcaccaagtctggcatcaagtgccagccatggagttccatgatccctcatgagcacagcttcctgccaagctcttaccggggaaaggatctgcaggagaactattgtagaaatcccagaggcgaggaaggaggaccctggtgttttaccagcaacccagaggtgcggtacgaggtgtgcgacataccccagtgcagcgaggtggaatgcatgacatgcaacggcgagagctaccggggcctgatggaccacacagagagcggcaaaatctgccaaagatgggatcaccagacccctcataggcacaagttcctgcccgagagataccctgacaagggcttcgacgacaattactgccggaaccctgatggacagcctagaccttggtgctacaccctggaccctcacaccagatgggaatactgcgccatcaagacatgtgccgataacaccatgaacgacaccgatgtgccactcgagacaactgagtgtatccagggccagggcgagggctacaggggcaccgtgaacaccatctggaacggcatcccttgtcagcggtgggacagccaatacccccacgaacatgatatgaccccagaaaacttcaagtgcaaagatctgcgggaaaactactgtagaaaccctgacggctccgagagcccttggtgcttcaccaccgaccctaacatcagggtgggctactgtagccagatccccaactgcgacatgagccacggtcaggactgctacagaggaaacggcaagaattacatgggcaacctgagccagaccagaagcggcctgacctgcagcatgtgggacaaaaacatggaagatctgcaccggcacatcttttgggagcctgacgccagcaagctgaatgagaactactgtcggaaccctgacgacgatgctcacggcccttggtgctacacaggcaaccctctgatcccttgggactattgtcctattagcaggtgtgaaggcgacacgacccctacaatcgtgaacctggatcacccagtgatcagctgtgctaaaacaaagcaactgagagtggtgaatggtatcccgacccggaccaacatcggatggatggtcagcctgcggtacagaaacaagcacatctgcggcggtagcctgatcaaggaatcctgggtgttgacagccagacagtgttttcccagcagagatctgaaggactacgaggcctggctgggcatccacgacgtgcacggcagaggcgacgagaagtgcaagcaggttctgaacgtgtcccagctggtgtacggccccgagggctctgatctggttctgatgaagcttgctagacccgctgtgctggatgacttcgtgtccaccatcgacctgccaaattacggatgtacaattcctgaaaagacctcctgttctgtgtacggctggggctacaccggactcatcaactatgacggcctgctgagagtggcccacctgtatatcatgggcaacgagaagtgcagccagcaccatagaggcaaggtgaccctgaacgagtctgaaatctgcgccggagccgagaaaatcggatctggcccctgcgaaggagattacggcggccctctggtctgcgagcagcacaagatgagaatggtgctgggcgtgatcgtgcccggcagaggctgcgccatccctaaccggcctggaatcttcgtgcgcgtggcctattacgccaaatggatccacaaaatcatcctgacatacaaggtcccacagtcttgataataggctggagcctcggtggccatgcttcttgccccttgggcctccccccagcccctcctccccttcctgcacccgtacccccgtggtctttgaataaagtctgagtgggcggcctcgagccgcggaaaaaaaaaaaaaaaaaaaaaaaaaaaaaagcatatgactaaaaaaaaaaaaaaaaaaaaaaaaaaaaaaaaaaaaaaaaaaaaaaaaaaaaaaaaaaaaaaaaaaaaaagtttaaacatttaaattctaga

SEQ ID NO: 115 - DNA, 2638 bp, synthetic construct
  source 1..2638: mol_type = other DNA; note; note (original language) = ACTG1 5'UTR-hHGF-CTSB 3'UTR-A30L70 (A1B12-hHGF-OS2)
ctctcgcactctgttcttccgccgctccgccgtcgcgtttctctgccggtcgcagctagcgccaccatgtgggtcaccaaactgctgcccgccctgctgctgcagcacgtgctcctgcacctgctgctgctgcctatcgccatcccttacgccgaaggccagagaaagcggagaaataccattcacgaatttaagaagagcgccaagaccacactgatcaagatcgaccctgccctgaaaatcaagaccaagaaagtgaacacagccgaccaatgcgctaatagatgcacaagaaacaaaggcctgcctttcacctgcaaggccttcgtgttcgataaggccagaaagcagtgcctgtggttccccttcaacagcatgagcagcggcgtgaagaaagaattcggtcacgagttcgacctgtacgagaataaggactacattagaaactgcatcatcggcaagggccggagctacaagggcaccgtgagcatcaccaagtctggcatcaagtgccagccatggagttccatgatccctcatgagcacagcttcctgccaagctcttaccggggaaaggatctgcaggagaactattgtagaaatcccagaggcgaggaaggaggaccctggtgttttaccagcaacccagaggtgcggtacgaggtgtgcgacataccccagtgcagcgaggtggaatgcatgacatgcaacggcgagagctaccggggcctgatggaccacacagagagcggcaaaatctgccaaagatgggatcaccagacccctcataggcacaagttcctgcccgagagataccctgacaagggcttcgacgacaattactgccggaaccctgatggacagcctagaccttggtgctacaccctggaccctcacaccagatgggaatactgcgccatcaagacatgtgccgataacaccatgaacgacaccgatgtgccactcgagacaactgagtgtatccagggccagggcgagggctacaggggcaccgtgaacaccatctggaacggcatcccttgtcagcggtgggacagccaatacccccacgaacatgatatgaccccagaaaacttcaagtgcaaagatctgcgggaaaactactgtagaaaccctgacggctccgagagcccttggtgcttcaccaccgaccctaacatcagggtgggctactgtagccagatccccaactgcgacatgagccacggtcaggactgctacagaggaaacggcaagaattacatgggcaacctgagccagaccagaagcggcctgacctgcagcatgtgggacaaaaacatggaagatctgcaccggcacatcttttgggagcctgacgccagcaagctgaatgagaactactgtcggaaccctgacgacgatgctcacggcccttggtgctacacaggcaaccctctgatcccttgggactattgtcctattagcaggtgtgaaggcgacacgacccctacaatcgtgaacctggatcacccagtgatcagctgtgctaaaacaaagcaactgagagtggtgaatggtatcccgacccggaccaacatcggatggatggtcagcctgcggtacagaaacaagcacatctgcggcggtagcctgatcaaggaatcctgggtgttgacagccagacagtgttttcccagcagagatctgaaggactacgaggcctggctgggcatccacgacgtgcacggcagaggcgacgagaagtgcaagcaggttctgaacgtgtcccagctggtgtacggccccgagggctctgatctggttctgatgaagcttgctagacccgctgtgctggatgacttcgtgtccaccatcgacctgccaaattacggatgtacaattcctgaaaagacctcctgttctgtgtacggctggggctacaccggactcatcaactatgacggcctgctgagagtggcccacctgtatatcatgggcaacgagaagtgcagccagcaccatagaggcaaggtgaccctgaacgagtctgaaatctgcgccggagccgagaaaatcggatctggcccctgcgaaggagattacggcggccctctggtctgcgagcagcacaagatgagaatggtgctgggcgtgatcgtgcccggcagaggctgcgccatccctaaccggcctggaatcttcgtgcgcgtggcctattacgccaaatggatccacaaaatcatcctgacatacaaggtcccacagtcttgataagggcccaccggttctgccgtgggcctgtcgtgccagtcctgggggcgagatcgggagaatcacgtcctggaactgcatgttcttgcgactcttgggacttcatcttaacttctcgctgccccagccatgttttcaaccatggcatccctcccccaattagttccctgtcatcctcgtcaaccttctctgtaagtgcctggtaagcttgcccttgcttaagaactcaaaacatagctgtgctctaccgcggaaaaaaaaaaaaaaaaaaaaaaaaaaaaaagcatatgactaaaaaaaaaaaaaaaaaaaaaaaaaaaaaaaaaaaaaaaaaaaaaaaaaaaaaaaaaaaaaaaaaaaaaagtttaaacatttaaattctaga

SEQ ID NO: 116 - DNA, 2652 bp, synthetic construct
  source 1..2652: mol_type = other DNA; note; note (original language) = CHCHD10 5'UTR-hHGF-CTSB 3'UTR-A30L70 (A15B12-hHGF-OS2)
ggcatttgtccccgcgacagcaccgctgccgccgtctctaaggtcgcccgggtcccaccgccgccaccgctagcgccaccatgtgggtcaccaaactgctgcccgccctgctgctgcagcacgtgctcctgcacctgctgctgctgcctatcgccatcccttacgccgaaggccagagaaagcggagaaataccattcacgaatttaagaagagcgccaagaccacactgatcaagatcgaccctgccctgaaaatcaagaccaagaaagtgaacacagccgaccaatgcgctaatagatgcacaagaaacaaaggcctgcctttcacctgcaaggccttcgtgttcgataaggccagaaagcagtgcctgtggttccccttcaacagcatgagcagcggcgtgaagaaagaattcggtcacgagttcgacctgtacgagaataaggactacattagaaactgcatcatcggcaagggccggagctacaagggcaccgtgagcatcaccaagtctggcatcaagtgccagccatggagttccatgatccctcatgagcacagcttcctgccaagctcttaccggggaaaggatctgcaggagaactattgtagaaatcccagaggcgaggaaggaggaccctggtgttttaccagcaacccagaggtgcggtacgaggtgtgcgacataccccagtgcagcgaggtggaatgcatgacatgcaacggcgagagctaccggggcctgatggaccacacagagagcggcaaaatctgccaaagatgggatcaccagacccctcataggcacaagttcctgcccgagagataccctgacaagggcttcgacgacaattactgccggaaccctgatggacagcctagaccttggtgctacaccctggaccctcacaccagatgggaatactgcgccatcaagacatgtgccgataacaccatgaacgacaccgatgtgccactcgagacaactgagtgtatccagggccagggcgagggctacaggggcaccgtgaacaccatctggaacggcatcccttgtcagcggtgggacagccaatacccccacgaacatgatatgaccccagaaaacttcaagtgcaaagatctgcgggaaaactactgtagaaaccctgacggctccgagagcccttggtgcttcaccaccgaccctaacatcagggtgggctactgtagccagatccccaactgcgacatgagccacggtcaggactgctacagaggaaacggcaagaattacatgggcaacctgagccagaccagaagcggcctgacctgcagcatgtgggacaaaaacatggaagatctgcaccggcacatcttttgggagcctgacgccagcaagctgaatgagaactactgtcggaaccctgacgacgatgctcacggcccttggtgctacacaggcaaccctctgatcccttgggactattgtcctattagcaggtgtgaaggcgacacgacccctacaatcgtgaacctggatcacccagtgatcagctgtgctaaaacaaagcaactgagagtggtgaatggtatcccgacccggaccaacatcggatggatggtcagcctgcggtacagaaacaagcacatctgcggcggtagcctgatcaaggaatcctgggtgttgacagccagacagtgttttcccagcagagatctgaaggactacgaggcctggctgggcatccacgacgtgcacggcagaggcgacgagaagtgcaagcaggttctgaacgtgtcccagctggtgtacggccccgagggctctgatctggttctgatgaagcttgctagacccgctgtgctggatgacttcgtgtccaccatcgacctgccaaattacggatgtacaattcctgaaaagacctcctgttctgtgtacggctggggctacaccggactcatcaactatgacggcctgctgagagtggcccacctgtatatcatgggcaacgagaagtgcagccagcaccatagaggcaaggtgaccctgaacgagtctgaaatctgcgccggagccgagaaaatcggatctggcccctgcgaaggagattacggcggccctctggtctgcgagcagcacaagatgagaatggtgctgggcgtgatcgtgcccggcagaggctgcgccatccctaaccggcctggaatcttcgtgcgcgtggcctattacgccaaatggatccacaaaatcatcctgacatacaaggtcccacagtcttgataagggcccaccggttctgccgtgggcctgtcgtgccagtcctgggggcgagatcgggagaatcacgtcctggaactgcatgttcttgcgactcttgggacttcatcttaacttctcgctgccccagccatgttttcaaccatggcatccctcccccaattagttccctgtcatcctcgtcaaccttctctgtaagtgcctggtaagcttgcccttgcttaagaactcaaaacatagctgtgctctaccgcggaaaaaaaaaaaaaaaaaaaaaaaaaaaaaagcatatgactaaaaaaaaaaaaaaaaaaaaaaaaaaaaaaaaaaaaaaaaaaaaaaaaaaaaaaaaaaaaaaaaaaaaaagtttaaacatttaaattctaga

SEQ ID NO: 117 - protein, 462 aa, Homo sapiens
  source 1..462: note; note (original language) = PD-1抗体重链氨基酸序列
MEWSWVFLFFLSVTTGVHSEVQLVESGGGLVQPGGSLRLSCAASGFTFSSYMMSWVRQAPGKGLEWVATISGGGANTYYPDSVKGRFTISRDNAKNSLYLQMNSLRAEDTAVYYCARQLYYFDYWGQGTTVTVSSASTKGPSVFPLAPCSRSTSESTAALGCLVKDYFPEPVTVSWNSGALTSGVHTFPAVLQSSGLYSLSSVVTVPSSSLGTKTYTCNVDHKPSNTKVDKRVESKYGPPCPPCPAPEFLGGPSVFLFPPKPKDTLMISRTPEVTCVVVDVSQEDPEVQFNWYVDGVEVHNAKTKPREEQFNSTYRVVSVLTVLHQDWLNGKEYKCKVSNKGLPSSIEKTISKAKGQPREPQVYTLPPSQEEMTKNQVSLTCLVKGFYPSDIAVEWESNGQPENNYKTTPPVLDSDGSFFLYSRLTVDKSRWQEGNVFSCSVMHEALHNHYTQKSLSLSLGK

SEQ ID NO: 118 - protein, 234 aa, Homo sapiens
  source 1..234: note; note (original language) = PD-1抗体轻链氨基酸序列
MSVPTQVLGLLLLWLTDARCDIQMTQSPSSLSASVGDRVTITCLASQTIGTWLTWYQQKPGKAPKLLIYTATSLADGVPSRFSGSGSGTDFTLTISSLQPEDFATYYCQQVYSIPWTFGGGTKVEIKRTVAAPSVFIFPPSDEQLKSGTASVVCLLNNFYPREAKVQWKVDNALQSGNSQESVTEQDSKDSTYSLSSTLTLSKADYEKHKVYACEVTHQGLSSPVTKSFNRGEC

SEQ ID NO: 119 - DNA, 1386 bp, synthetic construct
  source 1..1386: mol_type = other DNA; note; note (original language) = PD-1抗体重链DNA序列
atggaatggtcctgggtgttcctgttcttcctgtccgtgaccaccggcgtgcactccgaagtgcagctggtggaatctggcggcggactggtgcagcctggcggatctctgagactgtcttgtgccgcctccggcttcaccttctccagctacatgatgagctgggtgcgacaggcccctggcaagggactggaatgggtggccacaatctctggcggaggcgccaacacctactaccccgactctgtgaagggccggttcaccatctctcgggacaacgccaagaactccctgtacctgcagatgaacagcctgcgggccgaggacaccgccgtgtactactgtgcccggcagctgtactacttcgactactggggccagggcaccaccgtgaccgtgtcctctgcttctaccaagggcccctccgtgttccctctggctccttgctccagatccacctccgagtccaccgctgctctgggctgcctcgtgaaggactacttccccgagcctgtgacagtgtcctggaactctggcgccctgacctctggcgtgcacacctttccagcagtgctgcagtcctccggcctgtactccctgtcctccgtcgtgacagtgccctccagctctctgggcaccaagacctacacctgtaacgtggaccacaagccctccaacaccaaggtggacaagagagtggaatctaagtacggccctccctgccccccttgtcctgcccctgaatttctgggcggaccctctgtgtttctgttccccccaaagcccaaggacaccctgatgatctcccggacccccgaagtgacctgcgtggtggtggatgtgtcccaggaagatcccgaggtgcagttcaattggtacgtggacggcgtggaagtgcacaatgccaagaccaagcctagagaggaacagttcaactccacctaccgggtggtgtccgtgctgaccgtgctgcatcaggactggctgaacggcaaagagtacaagtgcaaggtgtccaacaagggcctgcccagctccatcgaaaagaccatctccaaggccaagggccagccccgggaaccccaggtgtacacactgcctccaagccaggaagagatgaccaagaaccaggtgtccctgacctgcctcgtgaaaggcttctacccctccgatatcgccgtggaatgggagtccaacggccagcctgagaacaactacaagaccaccccccctgtgctggactccgacggctccttctttctgtactctcgcctgaccgtggacaagtcccggtggcaggaaggcaacgtgttctcctgcagcgtgatgcacgaggccctgcacaaccactacacccagaagtccctgtccctgtctctgggaaag

SEQ ID NO: 120 - DNA, 702 bp, synthetic construct
  source 1..702: mol_type = other DNA; note; note (original language) = PD-1抗体轻链DNA序列
atgtccgtgcctacccaggtgctgggactgctgctgctgtggctgaccgacgccagatgcgacatccagatgacccagtccccctccagcctgtctgcctctgtgggcgacagagtgaccatcacctgtctggcctcccagaccatcggcacctggctgacctggtatcagcagaagcctggcaaggcccccaagctgctgatctacaccgccaccagtctggccgatggcgtgccctctagattctccggctctggctctggcaccgactttaccctgaccatcagctccctgcagcccgaggacttcgccacctactactgccagcaggtgtactccatcccctggacctttggcggaggcaccaaggtggaaatcaagcggaccgtggccgctccctccgtgttcatcttcccaccttccgacgagcagctgaagtccggaaccgccagtgtcgtgtgcctgctgaacaacttctacccccgcgaggccaaggtgcagtggaaggtggacaacgccctgcagtccggcaactcccaggaatccgtgaccgagcaggactccaaggacagcacctactccctgtcctccaccctgaccctgtccaaggccgactacgagaagcacaaggtgtacgcctgcgaagtgacccaccagggcctgtctagccccgtgaccaagtctttcaaccggggcgagtgc

SEQ ID NO: 121 - RNA, 1386 nt, synthetic construct
  source 1..1386: mol_type = other RNA; note; note (original language) = PD-1抗体重链mRNA序列
atggaatggtcctgggtgttcctgttcttcctgtccgtgaccaccggcgtgcactccgaagtgcagctggtggaatctggcggcggactggtgcagcctggcggatctctgagactgtcttgtgccgcctccggcttcaccttctccagctacatgatgagctgggtgcgacaggcccctggcaagggactggaatgggtggccacaatctctggcggaggcgccaacacctactaccccgactctgtgaagggccggttcaccatctctcgggacaacgccaagaactccctgtacctgcagatgaacagcctgcgggccgaggacaccgccgtgtactactgtgcccggcagctgtactacttcgactactggggccagggcaccaccgtgaccgtgtcctctgcttctaccaagggcccctccgtgttccctctggctccttgctccagatccacctccgagtccaccgctgctctgggctgcctcgtgaaggactacttccccgagcctgtgacagtgtcctggaactctggcgccctgacctctggcgtgcacacctttccagcagtgctgcagtcctccggcctgtactccctgtcctccgtcgtgacagtgccctccagctctctgggcaccaagacctacacctgtaacgtggaccacaagccctccaacaccaaggtggacaagagagtggaatctaagtacggccctccctgccccccttgtcctgcccctgaatttctgggcggaccctctgtgtttctgttccccccaaagcccaaggacaccctgatgatctcccggacccccgaagtgacctgcgtggtggtggatgtgtcccaggaagatcccgaggtgcagttcaattggtacgtggacggcgtggaagtgcacaatgccaagaccaagcctagagaggaacagttcaactccacctaccgggtggtgtccgtgctgaccgtgctgcatcaggactggctgaacggcaaagagtacaagtgcaaggtgtccaacaagggcctgcccagctccatcgaaaagaccatctccaaggccaagggccagccccgggaaccccaggtgtacacactgcctccaagccaggaagagatgaccaagaaccaggtgtccctgacctgcctcgtgaaaggcttctacccctccgatatcgccgtggaatgggagtccaacggccagcctgagaacaactacaagaccaccccccctgtgctggactccgacggctccttctttctgtactctcgcctgaccgtggacaagtcccggtggcaggaaggcaacgtgttctcctgcagcgtgatgcacgaggccctgcacaaccactacacccagaagtccctgtccctgtctctgggaaag

SEQ ID NO: 122 - RNA, 702 nt, synthetic construct
  source 1..702: mol_type = other RNA; note; note (original language) = PD-1抗体轻链mRNA序列
atgtccgtgcctacccaggtgctgggactgctgctgctgtggctgaccgacgccagatgcgacatccagatgacccagtccccctccagcctgtctgcctctgtgggcgacagagtgaccatcacctgtctggcctcccagaccatcggcacctggctgacctggtatcagcagaagcctggcaaggcccccaagctgctgatctacaccgccaccagtctggccgatggcgtgccctctagattctccggctctggctctggcaccgactttaccctgaccatcagctccctgcagcccgaggacttcgccacctactactgccagcaggtgtactccatcccctggacctttggcggaggcaccaaggtggaaatcaagcggaccgtggccgctccctccgtgttcatcttcccaccttccgacgagcagctgaagtccggaaccgccagtgtcgtgtgcctgctgaacaacttctacccccgcgaggccaaggtgcagtggaaggtggacaacgccctgcagtccggcaactcccaggaatccgtgaccgagcaggactccaaggacagcacctactccctgtcctccaccctgaccctgtccaaggccgactacgagaagcacaaggtgtacgcctgcgaagtgacccaccagggcctgtctagccccgtgaccaagtctttcaaccggggcgagtgc

SEQ ID NO: 123 - DNA, 2478 bp, synthetic construct
  source 1..2478: mol_type = other DNA; note; note (original language) = 5'UTR-anti PD-1-a 球蛋白 3'UTR-A30L70 (Mod.- anti PD-1)
gggaaataagagagaaaagaagagtaagaagaaatataagagccaccatggaatggtcctgggtgttcctgttcttcctgtccgtgaccaccggcgtgcactccgaagtgcagctggtggaatctggcggcggactggtgcagcctggcggatctctgagactgtcttgtgccgcctccggcttcaccttctccagctacatgatgagctgggtgcgacaggcccctggcaagggactggaatgggtggccacaatctctggcggaggcgccaacacctactaccccgactctgtgaagggccggttcaccatctctcgggacaacgccaagaactccctgtacctgcagatgaacagcctgcgggccgaggacaccgccgtgtactactgtgcccggcagctgtactacttcgactactggggccagggcaccaccgtgaccgtgtcctctgcttctaccaagggcccctccgtgttccctctggctccttgctccagatccacctccgagtccaccgctgctctgggctgcctcgtgaaggactacttccccgagcctgtgacagtgtcctggaactctggcgccctgacctctggcgtgcacacctttccagcagtgctgcagtcctccggcctgtactccctgtcctccgtcgtgacagtgccctccagctctctgggcaccaagacctacacctgtaacgtggaccacaagccctccaacaccaaggtggacaagagagtggaatctaagtacggccctccctgccccccttgtcctgcccctgaatttctgggcggaccctctgtgtttctgttccccccaaagcccaaggacaccctgatgatctcccggacccccgaagtgacctgcgtggtggtggatgtgtcccaggaagatcccgaggtgcagttcaattggtacgtggacggcgtggaagtgcacaatgccaagaccaagcctagagaggaacagttcaactccacctaccgggtggtgtccgtgctgaccgtgctgcatcaggactggctgaacggcaaagagtacaagtgcaaggtgtccaacaagggcctgcccagctccatcgaaaagaccatctccaaggccaagggccagccccgggaaccccaggtgtacacactgcctccaagccaggaagagatgaccaagaaccaggtgtccctgacctgcctcgtgaaaggcttctacccctccgatatcgccgtggaatgggagtccaacggccagcctgagaacaactacaagaccaccccccctgtgctggactccgacggctccttctttctgtactctcgcctgaccgtggacaagtcccggtggcaggaaggcaacgtgttctcctgcagcgtgatgcacgaggccctgcacaaccactacacccagaagtccctgtccctgtctctgggaaaggccaccaacttctccctgctgaagcaggccggcgacgtggaggagaaccccggccccatgtccgtgcctacccaggtgctgggactgctgctgctgtggctgaccgacgccagatgcgacatccagatgacccagtccccctccagcctgtctgcctctgtgggcgacagagtgaccatcacctgtctggcctcccagaccatcggcacctggctgacctggtatcagcagaagcctggcaaggcccccaagctgctgatctacaccgccaccagtctggccgatggcgtgccctctagattctccggctctggctctggcaccgactttaccctgaccatcagctccctgcagcccgaggacttcgccacctactactgccagcaggtgtactccatcccctggacctttggcggaggcaccaaggtggaaatcaagcggaccgtggccgctccctccgtgttcatcttcccaccttccgacgagcagctgaagtccggaaccgccagtgtcgtgtgcctgctgaacaacttctacccccgcgaggccaaggtgcagtggaaggtggacaacgccctgcagtccggcaactcccaggaatccgtgaccgagcaggactccaaggacagcacctactccctgtcctccaccctgaccctgtccaaggccgactacgagaagcacaaggtgtacgcctgcgaagtgacccaccagggcctgtctagccccgtgaccaagtctttcaaccggggcgagtgctgataagggcccaccggttgataataggctggagcctcggtggccatgcttcttgccccttgggcctccccccagcccctcctccccttcctgcacccgtacccccgtggtctttgaataaagtctgagtgggcggcctcgagccgcggaaaaaaaaaaaaaaaaaaaaaaaaaaaaaagcatatgactaaaaaaaaaaaaaaaaaaaaaaaaaaaaaaaaaaaaaaaaaaaaaaaaaaaaaaaaaaaaaaaaaaaaaattattgtttaaacatttaaattctaga

SEQ ID NO: 124 - DNA, 2602 bp, synthetic construct
  source 1..2602: mol_type = other DNA; note = ACTG1 5'UTR- anti PD-1-CTSB 3'UTR-A30L70 (A1B12- anti PD-1)
ctctcgcactctgttcttccgccgctccgccgtcgcgtttctctgccggtcgcaccaccatggaatggtcctgggtgttcctgttcttcctgtccgtgaccaccggcgtgcactccgaagtgcagctggtggaatctggcggcggactggtgcagcctggcggatctctgagactgtcttgtgccgcctccggcttcaccttctccagctacatgatgagctgggtgcgacaggcccctggcaagggactggaatgggtggccacaatctctggcggaggcgccaacacctactaccccgactctgtgaagggccggttcaccatctctcgggacaacgccaagaactccctgtacctgcagatgaacagcctgcgggccgaggacaccgccgtgtactactgtgcccggcagctgtactacttcgactactggggccagggcaccaccgtgaccgtgtcctctgcttctaccaagggcccctccgtgttccctctggctccttgctccagatccacctccgagtccaccgctgctctgggctgcctcgtgaaggactacttccccgagcctgtgacagtgtcctggaactctggcgccctgacctctggcgtgcacacctttccagcagtgctgcagtcctccggcctgtactccctgtcctccgtcgtgacagtgccctccagctctctgggcaccaagacctacacctgtaacgtggaccacaagccctccaacaccaaggtggacaagagagtggaatctaagtacggccctccctgccccccttgtcctgcccctgaatttctgggcggaccctctgtgtttctgttccccccaaagcccaaggacaccctgatgatctcccggacccccgaagtgacctgcgtggtggtggatgtgtcccaggaagatcccgaggtgcagttcaattggtacgtggacggcgtggaagtgcacaatgccaagaccaagcctagagaggaacagttcaactccacctaccgggtggtgtccgtgctgaccgtgctgcatcaggactggctgaacggcaaagagtacaagtgcaaggtgtccaacaagggcctgcccagctccatcgaaaagaccatctccaaggccaagggccagccccgggaaccccaggtgtacacactgcctccaagccaggaagagatgaccaagaaccaggtgtccctgacctgcctcgtgaaaggcttctacccctccgatatcgccgtggaatgggagtccaacggccagcctgagaacaactacaagaccaccccccctgtgctggactccgacggctccttctttctgtactctcgcctgaccgtggacaagtcccggtggcaggaaggcaacgtgttctcctgcagcgtgatgcacgaggccctgcacaaccactacacccagaagtccctgtccctgtctctgggaaaggccaccaacttctccctgctgaagcaggccggcgacgtggaggagaaccccggccccatgtccgtgcctacccaggtgctgggactgctgctgctgtggctgaccgacgccagatgcgacatccagatgacccagtccccctccagcctgtctgcctctgtgggcgacagagtgaccatcacctgtctggcctcccagaccatcggcacctggctgacctggtatcagcagaagcctggcaaggcccccaagctgctgatctacaccgccaccagtctggccgatggcgtgccctctagattctccggctctggctctggcaccgactttaccctgaccatcagctccctgcagcccgaggacttcgccacctactactgccagcaggtgtactccatcccctggacctttggcggaggcaccaaggtggaaatcaagcggaccgtggccgctccctccgtgttcatcttcccaccttccgacgagcagctgaagtccggaaccgccagtgtcgtgtgcctgctgaacaacttctacccccgcgaggccaaggtgcagtggaaggtggacaacgccctgcagtccggcaactcccaggaatccgtgaccgagcaggactccaaggacagcacctactccctgtcctccaccctgaccctgtccaaggccgactacgagaagcacaaggtgtacgcctgcgaagtgacccaccagggcctgtctagccccgtgaccaagtctttcaaccggggcgagtgctgataagggcccaccggtctgccgtgggcctgtcgtgccagtcctgggggcgagatcgggagaatcacgtcctggaactgcatgttcttgcgactcttgggacttcatcttaacttctcgctgccccagccatgttttcaaccatggcatccctcccccaattagttccctgtcatcctcgtcaaccttctctgtaagtgcctggtaagcttgcccttgcttaagaactcaaaacatagctgtgctctactcgagccgcggaaaaaaaaaaaaaaaaaaaaaaaaaaaaaagcatatgactaaaaaaaaaaaaaaaaaaaaaaaaaaaaaaaaaaaaaaaaaaaaaaaaaaaaaaaaaaaaaaaaaaaaaattattgtttaaacatttaaattctaga

SEQ ID NO: 125 - DNA, 2611 bp, synthetic construct
  source 1..2611: mol_type = other DNA; note = CHCHD10 5'UTR- anti PD-1-CTSB 3'UTR-A30L70 (A15B12- anti PD-1)
ggcatttgtccccgcgacagcaccgctgccgccgtctctaaggtcgcccgggtcccaccgccgccaccatggaatggtcctgggtgttcctgttcttcctgtccgtgaccaccggcgtgcactccgaagtgcagctggtggaatctggcggcggactggtgcagcctggcggatctctgagactgtcttgtgccgcctccggcttcaccttctccagctacatgatgagctgggtgcgacaggcccctggcaagggactggaatgggtggccacaatctctggcggaggcgccaacacctactaccccgactctgtgaagggccggttcaccatctctcgggacaacgccaagaactccctgtacctgcagatgaacagcctgcgggccgaggacaccgccgtgtactactgtgcccggcagctgtactacttcgactactggggccagggcaccaccgtgaccgtgtcctctgcttctaccaagggcccctccgtgttccctctggctccttgctccagatccacctccgagtccaccgctgctctgggctgcctcgtgaaggactacttccccgagcctgtgacagtgtcctggaactctggcgccctgacctctggcgtgcacacctttccagcagtgctgcagtcctccggcctgtactccctgtcctccgtcgtgacagtgccctccagctctctgggcaccaagacctacacctgtaacgtggaccacaagccctccaacaccaaggtggacaagagagtggaatctaagtacggccctccctgccccccttgtcctgcccctgaatttctgggcggaccctctgtgtttctgttccccccaaagcccaaggacaccctgatgatctcccggacccccgaagtgacctgcgtggtggtggatgtgtcccaggaagatcccgaggtgcagttcaattggtacgtggacggcgtggaagtgcacaatgccaagaccaagcctagagaggaacagttcaactccacctaccgggtggtgtccgtgctgaccgtgctgcatcaggactggctgaacggcaaagagtacaagtgcaaggtgtccaacaagggcctgcccagctccatcgaaaagaccatctccaaggccaagggccagccccgggaaccccaggtgtacacactgcctccaagccaggaagagatgaccaagaaccaggtgtccctgacctgcctcgtgaaaggcttctacccctccgatatcgccgtggaatgggagtccaacggccagcctgagaacaactacaagaccaccccccctgtgctggactccgacggctccttctttctgtactctcgcctgaccgtggacaagtcccggtggcaggaaggcaacgtgttctcctgcagcgtgatgcacgaggccctgcacaaccactacacccagaagtccctgtccctgtctctgggaaaggccaccaacttctccctgctgaagcaggccggcgacgtggaggagaaccccggccccatgtccgtgcctacccaggtgctgggactgctgctgctgtggctgaccgacgccagatgcgacatccagatgacccagtccccctccagcctgtctgcctctgtgggcgacagagtgaccatcacctgtctggcctcccagaccatcggcacctggctgacctggtatcagcagaagcctggcaaggcccccaagctgctgatctacaccgccaccagtctggccgatggcgtgccctctagattctccggctctggctctggcaccgactttaccctgaccatcagctccctgcagcccgaggacttcgccacctactactgccagcaggtgtactccatcccctggacctttggcggaggcaccaaggtggaaatcaagcggaccgtggccgctccctccgtgttcatcttcccaccttccgacgagcagctgaagtccggaaccgccagtgtcgtgtgcctgctgaacaacttctacccccgcgaggccaaggtgcagtggaaggtggacaacgccctgcagtccggcaactcccaggaatccgtgaccgagcaggactccaaggacagcacctactccctgtcctccaccctgaccctgtccaaggccgactacgagaagcacaaggtgtacgcctgcgaagtgacccaccagggcctgtctagccccgtgaccaagtctttcaaccggggcgagtgctgataagggcccaccggtctgccgtgggcctgtcgtgccagtcctgggggcgagatcgggagaatcacgtcctggaactgcatgttcttgcgactcttgggacttcatcttaacttctcgctgccccagccatgttttcaaccatggcatccctcccccaattagttccctgtcatcctcgtcaaccttctctgtaagtgcctggtaagcttgcccttgcttaagaactcaaaacatagctgtgctctactcgagccgcggaaaaaaaaaaaaaaaaaaaaaaaaaaaaaagcatatgactaaaaaaaaaaaaaaaaaaaaaaaaaaaaaaaaaaaaaaaaaaaaaaaaaaaaaaaaaaaaaaaaaaaaaattattgtttaaacatttaaattctaga

SEQ ID NO: 126 - DNA, 1653 bp, synthetic construct
  source 1..1653: mol_type = other DNA; note; note (original language) = 萤火虫荧光素酶核苷酸序列(Firefly Luciferase，Fluc)
atggaagacgccaaaaacataaagaaaggcccggcgccattctatccgctggaagatggaaccgctggagagcaactgcataaggctatgaagagatacgccctggttcctggaacaattgcttttacagatgcacatatcgaggtggacatcacttacgctgagtacttcgaaatgtccgttcggttggcagaagctatgaaacgatatgggctgaatacaaatcacagaatcgtcgtatgcagtgaaaactctcttcaattctttatgccggtgttgggcgcgttatttatcggagttgcagttgcgcccgcgaacgacatttataatgaacgtgaattgctcaacagtatgggcatttcgcagcctaccgtggtgttcgtttccaaaaaggggttgcaaaaaattttgaacgtgcaaaaaaagctcccaatcatccaaaaaattattatcatggattctaaaacggattaccagggatttcagtcgatgtacacgttcgtcacatctcatctacctcccggttttaatgaatacgattttgtgccagagtccttcgatagggacaagacaattgcactgatcatgaactcctctggatctactggtctgcctaaaggtgtcgctctgcctcatagaactgcctgcgtgagattctcgcatgccagagatcctatttttggcaatcaaatcattccggatactgcgattttaagtgttgttccattccatcacggttttggaatgtttactacactcggatatttgatatgtggatttcgagtcgtcttaatgtatagatttgaagaagagctgtttctgaggagccttcaggattacaagattcaaagtgcgctgctggtgccaaccctattctccttcttcgccaaaagcactctgattgacaaatacgatttatctaatttacacgaaattgcttctggtggcgctcccctctctaaggaagtcggggaagcggttgccaagaggttccatctgccaggtatcaggcaaggatatgggctcactgagactacatcagctattctgattacacccgagggggatgataaaccgggcgcggtcggtaaagttgttccattttttgaagcgaaggttgtggatctggataccgggaaaacgctgggcgttaatcaaagaggcgaactgtgtgtgagaggtcctatgattatgtccggttatgtaaacaatccggaagcgaccaacgccttgattgacaaggatggatggctacattctggagacatagcttactgggacgaagacgaacacttcttcatcgttgaccgcctgaagtctctgattaagtacaaaggctatcaggtggctcccgctgaattggaatccatcttgctccaacaccccaacatcttcgacgcaggtgtcgcaggtcttcccgacgatgacgccggtgaacttcccgccgccgttgttgttttggagcacggaaagacgatgacggaaaaagagatcgtggattacgtcgccagtcaagtaacaaccgcgaaaaagttgcgcggaggagttgtgtttgtggacgaagtaccgaaaggtcttaccggaaaactcgacgcaagaaaaatcagagagatcctcataaaggccaagaagggcggaaagatcgccgtgtaa

SEQ ID NO: 127 - DNA, 2630 bp, synthetic construct
  source 1..2630: mol_type = other DNA; note; note (original language) = HGF-OS2表达载体CHCHD10 5'UTR- hHGF-CTSB 3'UTR-A30L70（A16B12-HGF-OS2）
ccgctgccgccgtctctaaggtcgcccgggtcccaccgccgccaccgctagcgccaccatgtgggtcaccaaactgctgcccgccctgctgctgcagcacgtgctcctgcacctgctgctgctgcctatcgccatcccttacgccgaaggccagagaaagcggagaaataccattcacgaatttaagaagagcgccaagaccacactgatcaagatcgaccctgccctgaaaatcaagaccaagaaagtgaacacagccgaccaatgcgctaatagatgcacaagaaacaaaggcctgcctttcacctgcaaggccttcgtgttcgataaggccagaaagcagtgcctgtggttccccttcaacagcatgagcagcggcgtgaagaaagaattcggtcacgagttcgacctgtacgagaataaggactacattagaaactgcatcatcggcaagggccggagctacaagggcaccgtgagcatcaccaagtctggcatcaagtgccagccatggagttccatgatccctcatgagcacagcttcctgccaagctcttaccggggaaaggatctgcaggagaactattgtagaaatcccagaggcgaggaaggaggaccctggtgttttaccagcaacccagaggtgcggtacgaggtgtgcgacataccccagtgcagcgaggtggaatgcatgacatgcaacggcgagagctaccggggcctgatggaccacacagagagcggcaaaatctgccaaagatgggatcaccagacccctcataggcacaagttcctgcccgagagataccctgacaagggcttcgacgacaattactgccggaaccctgatggacagcctagaccttggtgctacaccctggaccctcacaccagatgggaatactgcgccatcaagacatgtgccgataacaccatgaacgacaccgatgtgccactcgagacaactgagtgtatccagggccagggcgagggctacaggggcaccgtgaacaccatctggaacggcatcccttgtcagcggtgggacagccaatacccccacgaacatgatatgaccccagaaaacttcaagtgcaaagatctgcgggaaaactactgtagaaaccctgacggctccgagagcccttggtgcttcaccaccgaccctaacatcagggtgggctactgtagccagatccccaactgcgacatgagccacggtcaggactgctacagaggaaacggcaagaattacatgggcaacctgagccagaccagaagcggcctgacctgcagcatgtgggacaaaaacatggaagatctgcaccggcacatcttttgggagcctgacgccagcaagctgaatgagaactactgtcggaaccctgacgacgatgctcacggcccttggtgctacacaggcaaccctctgatcccttgggactattgtcctattagcaggtgtgaaggcgacacgacccctacaatcgtgaacctggatcacccagtgatcagctgtgctaaaacaaagcaactgagagtggtgaatggtatcccgacccggaccaacatcggatggatggtcagcctgcggtacagaaacaagcacatctgcggcggtagcctgatcaaggaatcctgggtgttgacagccagacagtgttttcccagcagagatctgaaggactacgaggcctggctgggcatccacgacgtgcacggcagaggcgacgagaagtgcaagcaggttctgaacgtgtcccagctggtgtacggccccgagggctctgatctggttctgatgaagcttgctagacccgctgtgctggatgacttcgtgtccaccatcgacctgccaaattacggatgtacaattcctgaaaagacctcctgttctgtgtacggctggggctacaccggactcatcaactatgacggcctgctgagagtggcccacctgtatatcatgggcaacgagaagtgcagccagcaccatagaggcaaggtgaccctgaacgagtctgaaatctgcgccggagccgagaaaatcggatctggcccctgcgaaggagattacggcggccctctggtctgcgagcagcacaagatgagaatggtgctgggcgtgatcgtgcccggcagaggctgcgccatccctaaccggcctggaatcttcgtgcgcgtggcctattacgccaaatggatccacaaaatcatcctgacatacaaggtcccacagtcttgataagggcccaccggttctgccgtgggcctgtcgtgccagtcctgggggcgagatcgggagaatcacgtcctggaactgcatgttcttgcgactcttgggacttcatcttaacttctcgctgccccagccatgttttcaaccatggcatccctcccccaattagttccctgtcatcctcgtcaaccttctctgtaagtgcctggtaagcttgcccttgcttaagaactcaaaacatagctgtgctctaccgcggaaaaaaaaaaaaaaaaaaaaaaaaaaaaaagcatatgactaaaaaaaaaaaaaaaaaaaaaaaaaaaaaaaaaaaaaaaaaaaaaaaaaaaaaaaaaaaaaaaaaaaaaagtttaaacatttaaattctaga

SEQ ID NO: 128 - RNA, 2187 nt, synthetic construct
  source 1..2187: mol_type = other RNA; note; note (original language) = hHGF蛋白的mRNA序列
atgtgggtgaccaaactcctgccagccctgctgctgcagcatgtcctcctgcatctcctcctgctccccatcgccatcccctatgcagagggacaaaggaaaagaagaaatacaattcatgaattcaaaaaatcagcaaagactaccctaatcaaaatagatccagcactgaagataaaaaccaaaaaagtgaatactgcagaccaatgtgctaatagatgtactaggaataaaggacttccattcacttgcaaggcttttgtttttgataaagcaagaaaacaatgcctctggttccccttcaatagcatgtcaagtggagtgaaaaaagaatttggccatgaatttgacctctatgaaaacaaagactacattagaaactgcatcattggtaaaggacgcagctacaagggaacagtatctatcactaagagtggcatcaaatgtcagccctggagttccatgataccacacgaacacagctttttgccttcgagctatcggggtaaagacctacaggaaaactactgtcgaaatcctcgaggggaagaagggggaccctggtgtttcacaagcaatccagaggtacgctacgaagtctgtgacattcctcagtgttcagaagttgaatgcatgacctgcaatggggagagttatcgaggtctcatggatcatacagaatcaggcaagatttgtcagcgctgggatcatcagacaccacaccggcacaaattcttgcctgaaagatatcccgacaagggctttgatgataattattgccgcaatcccgatggccagccgaggccatggtgctatactcttgaccctcacacccgctgggagtactgtgcaattaaaacatgcgctgacaatactatgaatgacactgatgttcctttggaaacaactgaatgcatccaaggtcaaggagaaggctacaggggcactgtcaataccatttggaatggaattccatgtcagcgttgggattctcagtatcctcacgagcatgacatgactcctgaaaatttcaagtgcaaggacctacgagaaaattactgccgaaatccagatgggtctgaatcaccctggtgttttaccactgatccaaacatccgagttggctactgctcccaaattccaaactgtgatatgtcacatggacaagattgttatcgtgggaatggcaaaaattatatgggcaacttatcccaaacaagatctggactaacatgttcaatgtgggacaagaacatggaagacttacatcgtcatatcttctgggaaccagatgcaagtaagctgaatgagaattactgccgaaatccagatgatgatgctcatggaccctggtgctacacgggaaatccactcattccttgggattattgccctatttctcgttgtgaaggtgataccacacctacaatagtcaatttagaccatcccgtaatatcttgtgccaaaacgaaacaattgcgagttgtaaatgggattccaacacgaacaaacataggatggatggttagtttgagatacagaaataaacatatctgcggaggatcattgataaaggagagttgggttcttactgcacgacagtgtttcccttctcgagacttgaaagattatgaagcttggcttggaattcatgatgtccacggaagaggagatgagaaatgcaaacaggttctcaatgtttcccagctggtatatggccctgaaggatcagatctggttttaatgaagcttgccaggcctgctgtcctggatgattttgttagtacgattgatttacctaattatggatgcacaattcctgaaaagaccagttgcagtgtttatggctggggctacactggattgatcaactatgatggcctattacgagtggcacatctctatataatgggaaatgagaaatgcagccagcatcatcgagggaaggtgactctgaatgagtctgaaatatgtgctggggctgaaaagattggatcaggaccatgtgagggggattatggtggcccacttgtttgtgagcaacataaaatgagaatggttcttggtgtcattgttcctggtcgtggatgtgccattccaaatcgtcctggtatttttgtccgagtagcatattatgcaaaatggatacacaaaattattttaacatataaggtaccacagtcatag

SEQ ID NO: 129 - RNA, 2187 nt, synthetic construct
  source 1..2187: mol_type = other RNA; note; note (original language) = hHGF密码子优化mRNA序列1(hHGF-OS1)
atgtgggtgaccaaactgctccccgctctgctgctgcagcatgtgctgctccacctgctgctgctgccaatcgccatcccctacgctgaaggacagcggaagcgcagaaacacaattcacgaattcaagaagtccgccaaaacaacactgatcaagatcgaccctgccctgaaaatcaaaaccaagaaggtgaacactgccgatcagtgcgccaacagatgcacaagaaacaaaggcctgcccttcacatgcaaggcctttgtgttcgacaaggccagaaagcagtgcctgtggttccctttcaacagcatgagctctggcgtgaagaaagagttcggccacgaattcgacctgtacgagaacaaggattacatcagaaattgtatcatcggcaagggcagaagctacaaaggcacagtgtccatcaccaaaagcggcattaagtgtcagccttggagcagcatgatccctcacgagcacagcttcctgcctagctcttacagaggcaaggacctgcaggagaattactgccggaaccctagaggcgaggaaggcggcccttggtgctttaccagcaaccctgaggtgcggtacgaggtgtgtgacatcccccagtgcagcgaagtggaatgcatgacctgtaatggcgagagctacagaggcctcatggaccatacagagagcggaaagatttgtcaaagatgggatcaccagacacctcacagacacaaattcctgcccgaaagatatcctgacaagggcttcgacgacaactactgcagaaatcctgatggccaacccagaccttggtgctacaccctggatcctcataccagatgggagtactgtgccatcaagacctgcgctgataataccatgaacgacaccgatgtgcctctggaaacaaccgagtgcatccagggacagggcgaaggctaccggggcaccgtgaacaccatctggaacggcatcccctgccagagatgggacagccagtacccccacgaacacgatatgacccctgagaacttcaagtgcaaggacctgagagaaaattactgcagaaacccagacggaagcgagtctccttggtgttttaccaccgaccccaacatccgggtgggttactgcagccaaatccccaattgcgacatgagccacggccaggactgctaccggggaaacggcaaaaactacatgggcaatctgagccagacccggagcggtctgacctgctccatgtgggataagaacatggaagatctgcaccggcacatcttctgggagcctgacgcttctaagctgaacgagaactactgtaggaacccagacgacgatgcccacggtccctggtgctacaccggcaacccgctgatcccttgggactattgtcctatcagccgctgcgagggcgatacaacacctaccatcgtgaacctggaccaccctgtgatctcttgcgccaagaccaagcagctgagagtggtgaacggcatcccaacacggaccaacatcggatggatggtctccctgagataccggaacaagcacatctgcggcggctctctgatcaaggaatcttgggtcctgaccgccagacagtgcttccccagccgggacctgaaggactatgaggcctggctgggaatccacgacgtgcacggcagaggcgacgagaagtgcaagcaagtgctgaacgtgtcccagctggtgtacggccctgagggatctgatctggtcctgatgaaactggccagacccgccgtgctggacgactttgtgtccaccatcgacctgcctaactacggctgcaccatccctgaaaagaccagctgcagcgtgtacggctggggctatacaggcctgatcaactacgacggtctgctgcgggttgctcacctgtacatcatgggcaacgagaagtgcagccagcaccacagaggaaaggttacacttaacgagagcgagatctgcgccggcgccgagaaaatcggctccggcccttgtgaaggcgactacggaggccctctggtgtgcgaacagcacaagatgagaatggtgctgggcgtgatcgtgcccggaagaggctgtgcaatccctaataggcccggcattttcgtgcgggtggcctactacgccaagtggatccacaagatcatcctgacgtacaaggtgcctcagagctga

SEQ ID NO: 130 - RNA, 2187 nt, synthetic construct
  source 1..2187: mol_type = other RNA; note; note (original language) = hHGF密码子优化mRNA序列2(hHGF-OS2)
atgtgggtcaccaaactgctgcccgccctgctgctgcagcacgtgctcctgcacctgctgctgctgcctatcgccatcccttacgccgaaggccagagaaagcggagaaataccattcacgaatttaagaagagcgccaagaccacactgatcaagatcgaccctgccctgaaaatcaagaccaagaaagtgaacacagccgaccaatgcgctaatagatgcacaagaaacaaaggcctgcctttcacctgcaaggccttcgtgttcgataaggccagaaagcagtgcctgtggttccccttcaacagcatgagcagcggcgtgaagaaagaattcggtcacgagttcgacctgtacgagaataaggactacattagaaactgcatcatcggcaagggccggagctacaagggcaccgtgagcatcaccaagtctggcatcaagtgccagccatggagttccatgatccctcatgagcacagcttcctgccaagctcttaccggggaaaggatctgcaggagaactattgtagaaatcccagaggcgaggaaggaggaccctggtgttttaccagcaacccagaggtgcggtacgaggtgtgcgacataccccagtgcagcgaggtggaatgcatgacatgcaacggcgagagctaccggggcctgatggaccacacagagagcggcaaaatctgccaaagatgggatcaccagacccctcataggcacaagttcctgcccgagagataccctgacaagggcttcgacgacaattactgccggaaccctgatggacagcctagaccttggtgctacaccctggaccctcacaccagatgggaatactgcgccatcaagacatgtgccgataacaccatgaacgacaccgatgtgccactcgagacaactgagtgtatccagggccagggcgagggctacaggggcaccgtgaacaccatctggaacggcatcccttgtcagcggtgggacagccaatacccccacgaacatgatatgaccccagaaaacttcaagtgcaaagatctgcgggaaaactactgtagaaaccctgacggctccgagagcccttggtgcttcaccaccgaccctaacatcagggtgggctactgtagccagatccccaactgcgacatgagccacggtcaggactgctacagaggaaacggcaagaattacatgggcaacctgagccagaccagaagcggcctgacctgcagcatgtgggacaaaaacatggaagatctgcaccggcacatcttttgggagcctgacgccagcaagctgaatgagaactactgtcggaaccctgacgacgatgctcacggcccttggtgctacacaggcaaccctctgatcccttgggactattgtcctattagcaggtgtgaaggcgacacgacccctacaatcgtgaacctggatcacccagtgatcagctgtgctaaaacaaagcaactgagagtggtgaatggtatcccgacccggaccaacatcggatggatggtcagcctgcggtacagaaacaagcacatctgcggcggtagcctgatcaaggaatcctgggtgttgacagccagacagtgttttcccagcagagatctgaaggactacgaggcctggctgggcatccacgacgtgcacggcagaggcgacgagaagtgcaagcaggttctgaacgtgtcccagctggtgtacggccccgagggctctgatctggttctgatgaagcttgctagacccgctgtgctggatgacttcgtgtccaccatcgacctgccaaattacggatgtacaattcctgaaaagacctcctgttctgtgtacggctggggctacaccggactcatcaactatgacggcctgctgagagtggcccacctgtatatcatgggcaacgagaagtgcagccagcaccatagaggcaaggtgaccctgaacgagtctgaaatctgcgccggagccgagaaaatcggatctggcccctgcgaaggagattacggcggccctctggtctgcgagcagcacaagatgagaatggtgctgggcgtgatcgtgcccggcagaggctgcgccatccctaaccggcctggaatcttcgtgcgcgtggcctattacgccaaatggatccacaaaatcatcctgacatacaaggtcccacagtcttga

SEQ ID NO: 131 - RNA, 2187 nt, synthetic construct
  source 1..2187: mol_type = other RNA; note; note (original language) = hHGF密码子优化mRNA序列3(hHGF-OS3)
atgtgggtgaccaagctgctgcccgccctgctcctgcagcacgtgctgctgcacctgctcctgctgcccatcgccatcccctacgccgaggggcagagaaagagaagaaacaccatccacgagttcaagaagagcgccaagaccaccctgatcaagatcgaccccgccctgaagatcaagaccaagaaggtgaacaccgccgatcagtgcgccaacagatgcacaagaaacaagggcctgcccttcacctgcaaggccttcgtgttcgacaaggctagaaagcagtgcctgtggttccccttcaacagcatgagcagcggcgtgaagaaggagttcggccacgagttcgacctgtacgagaacaaggactacatcagaaactgcatcatcggcaagggcagaagctacaagggcaccgtgagcatcaccaagagcggcatcaagtgtcagccctggagcagcatgatcccccatgagcacagcttcctgcctagcagctacagagggaaggacctgcaagagaactactgcagaaaccctagaggcgaggagggcggcccttggtgtttcacaagcaatcccgaggtgagatacgaggtgtgcgacatccctcagtgcagcgaggtggagtgcatgacctgcaacggcgaaagctatagaggcctgatggaccacaccgagagcggcaagatttgtcagcggtgggatcaccaaaccccccacagacacaagttcctgcccgagagataccccgacaagggcttcgacgacaattactgtagaaaccccgacgggcagcctagaccctggtgttacaccctggacccccacacaagatgggagtactgcgccatcaagacctgcgccgacaacaccatgaacgacaccgacgtgcccctggagaccaccgagtgcatccaaggccaaggcgagggctacagaggcaccgtgaacaccatctggaacggcattccctgtcagagatgggacagccaatacccccatgaacacgatatgacccccgagaacttcaagtgcaaggacctgagagagaactactgccggaaccccgatggcagcgaatccccttggtgcttcaccaccgaccccaacatcagagtgggctactgcagccaaatccccaactgcgacatgagccacggccaagactgttacagagggaacggcaagaactacatgggcaacctgagccaaacaagaagcggcctgacctgcagcatgtgggacaagaacatggaggacctgcacagacacatcttctgggagcccgacgctagcaagctgaacgagaactactgtcggaaccccgacgacgatgcccacggcccctggtgctacaccggcaaccccctgatcccctgggactactgccccatcagcagatgcgagggcgacaccacccccaccatcgtgaacctggaccaccccgtgatcagctgtgccaagaccaagcaactgagagtggtgaacggcatccccacaagaaccaacattggctggatggtgagcctgagatacagaaacaagcacatctgcggcggcagcctgatcaaggagagctgggtgctgaccgctagacagtgcttccctagcagagacctgaaggactacgaggcctggctgggcatccacgacgtgcacggcagaggcgacgagaagtgtaaacaagtgctgaacgtgagccaactggtgtacggccccgagggcagcgacctggtgctgatgaagctggctagacccgccgtgctggacgacttcgtgagcaccatcgacctgcccaactacggctgcaccatccccgagaagacaagctgcagcgtgtacggctggggctacaccggcctgatcaactacgacggcctgctgagagtggcccacctgtacatcatgggcaacgagaagtgcagccaacaccaccggggcaaagtgaccctgaacgagagcgagatctgcgccggggctgagaaaatcggcagcggcccctgcgagggggactacgggggccccctggtgtgcgagcagcacaagatgagaatggtgctgggcgtgatcgtgcccggcagaggctgcgccatccccaacagacccggcatcttcgtgagagtggcctactacgccaagtggatccacaagatcatcctgacctacaaggtgcctcagagctga